European Patent Specification EP 3 577 234 B1, published March 20, 2024. Title: ENHANCED IMMUNE CELL RECEPTOR SEQUENCING METHODS. Applicant: Ludwig Institute for Cancer Research Ltd. Application Not Yet Assigned. The sequence listing filed with the application follows.

SEQUENCE LISTING (360 sequences)

SEQ ID NO: 1 - DNA, 54 bp, Artificial Sequence
  Synthetic Polynucleotide
  misc_feature (21)..(24): n is a, c, g, or t
  misc_feature (26)..(29): n is a, c, g, or t
tgtaatacgactcactatagnnnntnnnncttctacaggagctccagatgaaag

SEQ ID NO: 2 - DNA, 54 bp, Artificial Sequence
  Synthetic Polynucleotide
  misc_feature (21)..(24): n is a, c, g, or t
  misc_feature (26)..(29): n is a, c, g, or t
tgtaatacgactcactatagnnnntnnnncttttgaaggagctccagatgaaag

SEQ ID NO: 3 - DNA, 51 bp, Artificial Sequence
  Synthetic Polynucleotide
  misc_feature (21)..(24): n is a, c, g, or t
  misc_feature (26)..(29): n is a, c, g, or t
tgtaatacgactcactatagnnnntnnnntgctcatcctccaggtgcggga

SEQ ID NO: 4 - DNA, 52 bp, Artificial Sequence
  Synthetic Polynucleotide
  misc_feature (21)..(24): n is a, c, g, or t
  misc_feature (26)..(29): n is a, c, g, or t
tgtaatacgactcactatagnnnntnnnngaagaaaccatctgcccttgtga

SEQ ID NO: 5 - DNA, 54 bp, Artificial Sequence
  Synthetic Polynucleotide
  misc_feature (21)..(24): n is a, c, g, or t
  misc_feature (26)..(29): n is a, c, g, or t
tgtaatacgactcactatagnnnntnnnncctgccccgggtttccctgagcgac

SEQ ID NO: 6 - DNA, 52 bp, Artificial Sequence
  Synthetic Polynucleotide
  misc_feature (21)..(24): n is a, c, g, or t
  misc_feature (26)..(29): n is a, c, g, or t
tgtaatacgactcactatagnnnntnnnntctctgcgcattgcagacaccca

SEQ ID NO: 7 - DNA, 52 bp, Artificial Sequence
  Synthetic Polynucleotide
  misc_feature (21)..(24): n is a, c, g, or t
  misc_feature (26)..(29): n is a, c, g, or t
tgtaatacgactcactatagnnnntnnnnttgtttcatatcacagcctccca

SEQ ID NO: 8 - DNA, 51 bp, Artificial Sequence
  Synthetic Polynucleotide
  misc_feature (21)..(24): n is a, c, g, or t
  misc_feature (26)..(29): n is a, c, g, or t
tgtaatacgactcactatagnnnntnnnngcttgtacattacagccgtgca

SEQ ID NO: 9 - DNA, 51 bp, Artificial Sequence
  Synthetic Polynucleotide
  misc_feature (21)..(24): n is a, c, g, or t
  misc_feature (26)..(29): n is a, c, g, or t
tgtaatacgactcactatagnnnntnnnnatctgaggaaaccctctgtgca

SEQ ID NO: 10 - DNA, 52 bp, Artificial Sequence
  Synthetic Polynucleotide
  misc_feature (21)..(24): n is a, c, g, or t
  misc_feature (26)..(29): n is a, c, g, or t
tgtaatacgactcactatagnnnntnnnnacctgacgaaaccctcagcccat

SEQ ID NO: 11 - DNA, 53 bp, Artificial Sequence
  Synthetic Polynucleotide
  misc_feature (21)..(24): n is a, c, g, or t
  misc_feature (26)..(29): n is a, c, g, or t
tgtaatacgactcactatagnnnntnnnncctatgcctgtctttactttaatc

SEQ ID NO: 12 - DNA, 53 bp, Artificial Sequence
  Synthetic Polynucleotide
  misc_feature (21)..(24): n is a, c, g, or t
  misc_feature (26)..(29): n is a, c, g, or t
tgtaatacgactcactatagnnnntnnnncttgaggaaaccctcagtccatat

SEQ ID NO: 13 - DNA, 53 bp, Artificial Sequence
  Synthetic Polynucleotide
  misc_feature (21)..(24): n is a, c, g, or t
  misc_feature (26)..(29): n is a, c, g, or t
tgtaatacgactcactatagnnnntnnnngaaaccatcaacccatgtgagtga

SEQ ID NO: 14 - DNA, 52 bp, Artificial Sequence
  Synthetic Polynucleotide
  misc_feature (21)..(24): n is a, c, g, or t
  misc_feature (26)..(29): n is a, c, g, or t
tgtaatacgactcactatagnnnntnnnnacttggagaaagactcagttcaa

SEQ ID NO: 15 - DNA, 52 bp, Artificial Sequence
  Synthetic Polynucleotide
  misc_feature (21)..(24): n is a, c, g, or t
  misc_feature (26)..(29): n is a, c, g, or t
tgtaatacgactcactatagnnnntnnnnacttggagaaaggctcagttcaa

SEQ ID NO: 16 - DNA, 49 bp, Artificial Sequence
  Synthetic Polynucleotide
  misc_feature (21)..(24): n is a, c, g, or t
  misc_feature (26)..(29): n is a, c, g, or t
tgtaatacgactcactatagnnnntnnnnctgcacatcacagcctccca

SEQ ID NO: 17 - DNA, 53 bp, Artificial Sequence
  Synthetic Polynucleotide
  misc_feature (21)..(24): n is a, c, g, or t
  misc_feature (26)..(29): n is a, c, g, or t
tgtaatacgactcactatagnnnntnnnngtttggaatatcgcagcctctcat

SEQ ID NO: 18 - DNA, 52 bp, Artificial Sequence
  Synthetic Polynucleotide
  misc_feature (21)..(24): n is a, c, g, or t
  misc_feature (26)..(29): n is a, c, g, or t
tgtaatacgactcactatagnnnntnnnnccctgctcatcagagactccaag

SEQ ID NO: 19 - DNA, 52 bp, Artificial Sequence
  Synthetic Polynucleotide
  misc_feature (21)..(24): n is a, c, g, or t
  misc_feature (26)..(29): n is a, c, g, or t
tgtaatacgactcactatagnnnntnnnnctctgctcatcagagactcccag

SEQ ID NO: 20 - DNA, 52 bp, Artificial Sequence
  Synthetic Polynucleotide
  misc_feature (21)..(24): n is a, c, g, or t
  misc_feature (26)..(29): n is a, c, g, or t
tgtaatacgactcactatagnnnntnnnnccttgttcatcagagactcacag

SEQ ID NO: 21 - DNA, 53 bp, Artificial Sequence
  Synthetic Polynucleotide
  misc_feature (21)..(24): n is a, c, g, or t
  misc_feature (26)..(29): n is a, c, g, or t
tgtaatacgactcactatagnnnntnnnntccctgcacatcacagagacccaa

SEQ ID NO: 22 - DNA, 53 bp, Artificial Sequence
  Synthetic Polynucleotide
  misc_feature (21)..(24): n is a, c, g, or t
  misc_feature (26)..(29): n is a, c, g, or t
tgtaatacgactcactatagnnnntnnnntctctgcaaattgcagctactcaa

SEQ ID NO: 23 - DNA, 53 bp, Artificial Sequence
  Synthetic Polynucleotide
  misc_feature (21)..(24): n is a, c, g, or t
  misc_feature (26)..(29): n is a, c, g, or t
tgtaatacgactcactatagnnnntnnnnttgtcatctccgcttcacaactgg

SEQ ID NO: 24 - DNA, 53 bp, Artificial Sequence
  Synthetic Polynucleotide
  misc_feature (21)..(24): n is a, c, g, or t
  misc_feature (26)..(29): n is a, c, g, or t
tgtaatacgactcactatagnnnntnnnngttttgaatatgctggtctctcat

SEQ ID NO: 25 - DNA, 53 bp, Artificial Sequence
  Synthetic Polynucleotide
  misc_feature (21)..(24): n is a, c, g, or t
  misc_feature (26)..(29): n is a, c, g, or t
tgtaatacgactcactatagnnnntnnnncctgaagaaaccatttgctcaaga

SEQ ID NO: 26 - DNA, 53 bp, Artificial Sequence
  Synthetic Polynucleotide
  misc_feature (21)..(24): n is a, c, g, or t
  misc_feature (26)..(29): n is a, c, g, or t
tgtaatacgactcactatagnnnntnnnntccttgttgatcacggcttcccgg

SEQ ID NO: 27 - DNA, 51 bp, Artificial Sequence
  Synthetic Polynucleotide
  misc_feature (21)..(24): n is a, c, g, or t
  misc_feature (26)..(29): n is a, c, g, or t
tgtaatacgactcactatagnnnntnnnnacctggagaagccctcggtgca

SEQ ID NO: 28 - DNA, 53 bp, Artificial Sequence
  Synthetic Polynucleotide
  misc_feature (21)..(24): n is a, c, g, or t
  misc_feature (26)..(29): n is a, c, g, or t
tgtaatacgactcactatagnnnntnnnncaccatcacagcctcacaagtcgt

SEQ ID NO: 29 - DNA, 51 bp, Artificial Sequence
  Synthetic Polynucleotide
  misc_feature (21)..(24): n is a, c, g, or t
  misc_feature (26)..(29): n is a, c, g, or t
tgtaatacgactcactatagnnnntnnnntttctgcacatcacagccccta

SEQ ID NO: 30 - DNA, 54 bp, Artificial Sequence
  Synthetic Polynucleotide
  misc_feature (21)..(24): n is a, c, g, or t
  misc_feature (26)..(29): n is a, c, g, or t
tgtaatacgactcactatagnnnntnnnnctttatacattgcagcttctcagcc

SEQ ID NO: 31 - DNA, 53 bp, Artificial Sequence
  Synthetic Polynucleotide
  misc_feature (21)..(24): n is a, c, g, or t
  misc_feature (26)..(29): n is a, c, g, or t
tgtaatacgactcactatagnnnntnnnngtacatttcctcttcccagaccac

SEQ ID NO: 32 - DNA, 53 bp, Artificial Sequence
  Synthetic Polynucleotide
  misc_feature (21)..(24): n is a, c, g, or t
  misc_feature (26)..(29): n is a, c, g, or t
tgtaatacgactcactatagnnnntnnnncattgcatatcatggattcccagc

SEQ ID NO: 33 - DNA, 53 bp, Artificial Sequence
  Synthetic Polynucleotide
  misc_feature (21)..(24): n is a, c, g, or t
  misc_feature (26)..(29): n is a, c, g, or t
tgtaatacgactcactatagnnnntnnnngctatttgtacatcaaaggatccc

SEQ ID NO: 34 - DNA, 52 bp, Artificial Sequence
  Synthetic Polynucleotide
  misc_feature (21)..(24): n is a, c, g, or t
  misc_feature (26)..(29): n is a, c, g, or t
tgtaatacgactcactatagnnnntnnnncagctccctgcacatcacagcca

SEQ ID NO: 35 - DNA, 54 bp, Artificial Sequence
  Synthetic Polynucleotide
  misc_feature (21)..(24): n is a, c, g, or t
  misc_feature (26)..(29): n is a, c, g, or t
tgtaatacgactcactatagnnnntnnnnttgatcctgccccacgctacgctga

SEQ ID NO: 36 - DNA, 54 bp, Artificial Sequence
  Synthetic Polynucleotide
  misc_feature (21)..(24): n is a, c, g, or t
  misc_feature (26)..(29): n is a, c, g, or t
tgtaatacgactcactatagnnnntnnnnttgatcctgcaccgtgctaccttga

SEQ ID NO: 37 - DNA, 52 bp, Artificial Sequence
  Synthetic Polynucleotide
  misc_feature (21)..(24): n is a, c, g, or t
  misc_feature (26)..(29): n is a, c, g, or t
tgtaatacgactcactatagnnnntnnnngttctctccacatcactgcagcc

SEQ ID NO: 38 - DNA, 52 bp, Artificial Sequence
  Synthetic Polynucleotide
  misc_feature (21)..(24): n is a, c, g, or t
  misc_feature (26)..(29): n is a, c, g, or t
tgtaatacgactcactatagnnnntnnnngccacctatacatcagattccca

SEQ ID NO: 39 - DNA, 52 bp, Artificial Sequence
  Synthetic Polynucleotide
  misc_feature (21)..(24): n is a, c, g, or t
  misc_feature (26)..(29): n is a, c, g, or t
tgtaatacgactcactatagnnnntnnnntctctgcacattgtgccctccca

SEQ ID NO: 40 - DNA, 54 bp, Artificial Sequence
  Synthetic Polynucleotide
  misc_feature (21)..(24): n is a, c, g, or t
  misc_feature (26)..(29): n is a, c, g, or t
tgtaatacgactcactatagnnnntnnnnccctgtaccttacggcctcccagct

SEQ ID NO: 41 - DNA, 53 bp, Artificial Sequence
  Synthetic Polynucleotide
  misc_feature (21)..(24): n is a, c, g, or t
  misc_feature (26)..(29): n is a, c, g, or t
tgtaatacgactcactatagnnnntnnnncttatcatatcatcatcacagcca

SEQ ID NO: 42 - DNA, 53 bp, Artificial Sequence
  Synthetic Polynucleotide
  misc_feature (21)..(24): n is a, c, g, or t
  misc_feature (26)..(29): n is a, c, g, or t
tgtaatacgactcactatagnnnntnnnntccctgcatattacagccacccaa

SEQ ID NO: 43 - DNA, 53 bp, Artificial Sequence
  Synthetic Polynucleotide
  misc_feature (21)..(24): n is a, c, g, or t
  misc_feature (26)..(29): n is a, c, g, or t
tgtaatacgactcactatagnnnntnnnnacctcaccatcaattccttaaaac

SEQ ID NO: 44 - DNA, 53 bp, Artificial Sequence
  Synthetic Polynucleotide
  misc_feature (21)..(24): n is a, c, g, or t
  misc_feature (26)..(29): n is a, c, g, or t
tgtaatacgactcactatagnnnntnnnntccctgcatatcacagcctcccag

SEQ ID NO: 45 - DNA, 53 bp, Artificial Sequence
  Synthetic Polynucleotide
  misc_feature (21)..(24): n is a, c, g, or t
  misc_feature (26)..(29): n is a, c, g, or t
tgtaatacgactcactatagnnnntnnnncttcctgaatatctcagcatccat

SEQ ID NO: 46 - DNA, 52 bp, Artificial Sequence
  Synthetic Polynucleotide
  misc_feature (21)..(24): n is a, c, g, or t
  misc_feature (26)..(29): n is a, c, g, or t
tgtaatacgactcactatagnnnntnnnntcctgaacatcacagccacccag

SEQ ID NO: 47 - DNA, 53 bp, Artificial Sequence
  Synthetic Polynucleotide
  misc_feature (21)..(24): n is a, c, g, or t
  misc_feature (26)..(29): n is a, c, g, or t
tgtaatacgactcactatagnnnntnnnntccctgcacatacaggattcccag

SEQ ID NO: 48 - DNA, 52 bp, Artificial Sequence
  Synthetic Polynucleotide
  misc_feature (21)..(24): n is a, c, g, or t
  misc_feature (26)..(29): n is a, c, g, or t
tgtaatacgactcactatagnnnntnnnncaagatctcagactcacagctgg

SEQ ID NO: 49 - DNA, 52 bp, Artificial Sequence
  Synthetic Polynucleotide
  misc_feature (21)..(24): n is a, c, g, or t
  misc_feature (26)..(29): n is a, c, g, or t
tgtaatacgactcactatagnnnntnnnnccgtctcagcaccctccacatca

SEQ ID NO: 50 - DNA, 53 bp, Artificial Sequence
  Synthetic Polynucleotide
  misc_feature (21)..(24): n is a, c, g, or t
  misc_feature (26)..(29): n is a, c, g, or t
tgtaatacgactcactatagnnnntnnnnccattgtgaaatattcagtccagg

SEQ ID NO: 51 - DNA, 52 bp, Artificial Sequence
  Synthetic Polynucleotide
  misc_feature (21)..(24): n is a, c, g, or t
  misc_feature (26)..(29): n is a, c, g, or t
tgtaatacgactcactatagnnnnannnngtggtcgcactgcagcaagaaga

SEQ ID NO: 52 - DNA, 53 bp, Artificial Sequence
  Synthetic Polynucleotide
  misc_feature (21)..(24): n is a, c, g, or t
  misc_feature (26)..(29): n is a, c, g, or t
tgtaatacgactcactatagnnnnannnngatccggtccacaaagctggagga

SEQ ID NO: 53 - DNA, 53 bp, Artificial Sequence
  Synthetic Polynucleotide
  misc_feature (21)..(24): n is a, c, g, or t
  misc_feature (26)..(29): n is a, c, g, or t
tgtaatacgactcactatagnnnnannnncatcaattccctggagcttggtga

SEQ ID NO: 54 - DNA, 53 bp, Artificial Sequence
  Synthetic Polynucleotide
  misc_feature (21)..(24): n is a, c, g, or t
  misc_feature (26)..(29): n is a, c, g, or t
tgtaatacgactcactatagnnnnannnnttcacctacacgccctgcagccag

SEQ ID NO: 55 - DNA, 53 bp, Artificial Sequence
  Synthetic Polynucleotide
  misc_feature (21)..(24): n is a, c, g, or t
  misc_feature (26)..(29): n is a, c, g, or t
tgtaatacgactcactatagnnnnannnnttcacctacacaccctgcagccag

SEQ ID NO: 56 - DNA, 52 bp, Artificial Sequence
  Synthetic Polynucleotide
  misc_feature (21)..(24): n is a, c, g, or t
  misc_feature (26)..(29): n is a, c, g, or t
tgtaatacgactcactatagnnnnannnngaatgtgagcaccttggagctgg

SEQ ID NO: 57 - DNA, 53 bp, Artificial Sequence
  Synthetic Polynucleotide
  misc_feature (21)..(24): n is a, c, g, or t
  misc_feature (26)..(29): n is a, c, g, or t
tgtaatacgactcactatagnnnnannnntactgagtcaaacacggagctagg

SEQ ID NO: 58 - DNA, 53 bp, Artificial Sequence
  Synthetic Polynucleotide
  misc_feature (21)..(24): n is a, c, g, or t
  misc_feature (26)..(29): n is a, c, g, or t
tgtaatacgactcactatagnnnnannnngctctgagatgaatgtgagtgcct

SEQ ID NO: 59 - DNA, 51 bp, Artificial Sequence
  Synthetic Polynucleotide
  misc_feature (21)..(24): n is a, c, g, or t
  misc_feature (26)..(29): n is a, c, g, or t
tgtaatacgactcactatagnnnnannnnctgagctgaatgtgaacgcctt

SEQ ID NO: 60 - DNA, 51 bp, Artificial Sequence
  Synthetic Polynucleotide
  misc_feature (21)..(24): n is a, c, g, or t
  misc_feature (26)..(29): n is a, c, g, or t
tgtaatacgactcactatagnnnnannnngagttctcgctcaggctggagt

SEQ ID NO: 61 - DNA, 51 bp, Artificial Sequence
  Synthetic Polynucleotide
  misc_feature (21)..(24): n is a, c, g, or t
  misc_feature (26)..(29): n is a, c, g, or t
tgtaatacgactcactatagnnnnannnnctggggttggagtcggctgctc

SEQ ID NO: 62 - DNA, 51 bp, Artificial Sequence
  Synthetic Polynucleotide
  misc_feature (21)..(24): n is a, c, g, or t
  misc_feature (26)..(29): n is a, c, g, or t
tgtaatacgactcactatagnnnnannnncccctcacgttggcgtctgctg

SEQ ID NO: 63 - DNA, 51 bp, Artificial Sequence
  Synthetic Polynucleotide
  misc_feature (21)..(24): n is a, c, g, or t
  misc_feature (26)..(29): n is a, c, g, or t
tgtaatacgactcactatagnnnnannnntcccgctcaggctgctgtcggc

SEQ ID NO: 64 - DNA, 51 bp, Artificial Sequence
  Synthetic Polynucleotide
  misc_feature (21)..(24): n is a, c, g, or t
  misc_feature (26)..(29): n is a, c, g, or t
tgtaatacgactcactatagnnnnannnngatttcccgctcaggctggagt

SEQ ID NO: 65 - DNA, 52 bp, Artificial Sequence
  Synthetic Polynucleotide
  misc_feature (21)..(24): n is a, c, g, or t
  misc_feature (26)..(29): n is a, c, g, or t
tgtaatacgactcactatagnnnnannnntccccctcaagctggagtcagct

SEQ ID NO: 66 - DNA, 51 bp, Artificial Sequence
  Synthetic Polynucleotide
  misc_feature (21)..(24): n is a, c, g, or t
  misc_feature (26)..(29): n is a, c, g, or t
tgtaatacgactcactatagnnnnannnntcccactcaggctggtgtcggc

SEQ ID NO: 67 - DNA, 51 bp, Artificial Sequence
  Synthetic Polynucleotide
  misc_feature (21)..(24): n is a, c, g, or t
  misc_feature (26)..(29): n is a, c, g, or t
tgtaatacgactcactatagnnnnannnnctctgaagttccagcgcacaca

SEQ ID NO: 68 - DNA, 51 bp, Artificial Sequence
  Synthetic Polynucleotide
  misc_feature (21)..(24): n is a, c, g, or t
  misc_feature (26)..(29): n is a, c, g, or t
tgtaatacgactcactatagnnnnannnngatccagcgcacacagcaggag

SEQ ID NO: 69 - DNA, 52 bp, Artificial Sequence
  Synthetic Polynucleotide
  misc_feature (21)..(24): n is a, c, g, or t
  misc_feature (26)..(29): n is a, c, g, or t
tgtaatacgactcactatagnnnnannnnactctgaagatccagcgcacaga

SEQ ID NO: 70 - DNA, 51 bp, Artificial Sequence
  Synthetic Polynucleotide
  misc_feature (21)..(24): n is a, c, g, or t
  misc_feature (26)..(29): n is a, c, g, or t
tgtaatacgactcactatagnnnnannnnagatccagcgcacagagcaagg

SEQ ID NO: 71 - DNA, 51 bp, Artificial Sequence
  Synthetic Polynucleotide
  misc_feature (21)..(24): n is a, c, g, or t
  misc_feature (26)..(29): n is a, c, g, or t
tgtaatacgactcactatagnnnnannnncagcgcacagagcagcgggact

SEQ ID NO: 72 - DNA, 51 bp, Artificial Sequence
  Synthetic Polynucleotide
  misc_feature (21)..(24): n is a, c, g, or t
  misc_feature (26)..(29): n is a, c, g, or t
tgtaatacgactcactatagnnnnannnngagatccagcgcacagagcagg

SEQ ID NO: 73 - DNA, 51 bp, Artificial Sequence
  Synthetic Polynucleotide
  misc_feature (21)..(24): n is a, c, g, or t
  misc_feature (26)..(29): n is a, c, g, or t
tgtaatacgactcactatagnnnnannnnccctcaaccctggagtctacta

SEQ ID NO: 74 - DNA, 51 bp, Artificial Sequence
  Synthetic Polynucleotide
  misc_feature (21)..(24): n is a, c, g, or t
  misc_feature (26)..(29): n is a, c, g, or t
tgtaatacgactcactatagnnnnannnntccccaatcctggcatccacca

SEQ ID NO: 75 - DNA, 52 bp, Artificial Sequence
  Synthetic Polynucleotide
  misc_feature (21)..(24): n is a, c, g, or t
  misc_feature (26)..(29): n is a, c, g, or t
tgtaatacgactcactatagnnnnannnnctaaacctgagctctctggagct

SEQ ID NO: 76 - DNA, 51 bp, Artificial Sequence
  Synthetic Polynucleotide
  misc_feature (21)..(24): n is a, c, g, or t
  misc_feature (26)..(29): n is a, c, g, or t
tgtaatacgactcactatagnnnnannnnccctcactctggagtctgctgc

SEQ ID NO: 77 - DNA, 51 bp, Artificial Sequence
  Synthetic Polynucleotide
  misc_feature (21)..(24): n is a, c, g, or t
  misc_feature (26)..(29): n is a, c, g, or t
tgtaatacgactcactatagnnnnannnnccctcactctggagtcagctac

SEQ ID NO: 78 - DNA, 51 bp, Artificial Sequence
  Synthetic Polynucleotide
  misc_feature (21)..(24): n is a, c, g, or t
  misc_feature (26)..(29): n is a, c, g, or t
tgtaatacgactcactatagnnnnannnntcctcactctggagtccgctac

SEQ ID NO: 79 - DNA, 52 bp, Artificial Sequence
  Synthetic Polynucleotide
  misc_feature (21)..(24): n is a, c, g, or t
  misc_feature (26)..(29): n is a, c, g, or t
tgtaatacgactcactatagnnnnannnnccactctcaagatccagcctgca

SEQ ID NO: 80 - DNA, 52 bp, Artificial Sequence
  Synthetic Polynucleotide
  misc_feature (21)..(24): n is a, c, g, or t
  misc_feature (26)..(29): n is a, c, g, or t
tgtaatacgactcactatagnnnnannnngaggatccagcccatggaaccca

SEQ ID NO: 81 - DNA, 51 bp, Artificial Sequence
  Synthetic Polynucleotide
  misc_feature (21)..(24): n is a, c, g, or t
  misc_feature (26)..(29): n is a, c, g, or t
tgtaatacgactcactatagnnnnannnnctgaagatccagcctgcagagc

SEQ ID NO: 82 - DNA, 51 bp, Artificial Sequence
  Synthetic Polynucleotide
  misc_feature (21)..(24): n is a, c, g, or t
  misc_feature (26)..(29): n is a, c, g, or t
tgtaatacgactcactatagnnnnannnncagccctcagaacccagggact

SEQ ID NO: 83 - DNA, 52 bp, Artificial Sequence
  Synthetic Polynucleotide
  misc_feature (21)..(24): n is a, c, g, or t
  misc_feature (26)..(29): n is a, c, g, or t
tgtaatacgactcactatagnnnnannnngagctccttggagctgggggact

SEQ ID NO: 84 - DNA, 51 bp, Artificial Sequence
  Synthetic Polynucleotide
  misc_feature (21)..(24): n is a, c, g, or t
  misc_feature (26)..(29): n is a, c, g, or t
tgtaatacgactcactatagnnnnannnnggtgcagcctgcagaactggag

SEQ ID NO: 85 - DNA, 51 bp, Artificial Sequence
  Synthetic Polynucleotide
  misc_feature (21)..(24): n is a, c, g, or t
  misc_feature (26)..(29): n is a, c, g, or t
tgtaatacgactcactatagnnnnannnngacatccgctcaccaggcctgg

SEQ ID NO: 86 - DNA, 51 bp, Artificial Sequence
  Synthetic Polynucleotide
  misc_feature (21)..(24): n is a, c, g, or t
  misc_feature (26)..(29): n is a, c, g, or t
tgtaatacgactcactatagnnnnannnntgagatccaggctacgaagctt

SEQ ID NO: 87 - DNA, 51 bp, Artificial Sequence
  Synthetic Polynucleotide
  misc_feature (21)..(24): n is a, c, g, or t
  misc_feature (26)..(29): n is a, c, g, or t
tgtaatacgactcactatagnnnnannnngaagatccatcccgcagagccg

SEQ ID NO: 88 - DNA, 51 bp, Artificial Sequence
  Synthetic Polynucleotide
  misc_feature (21)..(24): n is a, c, g, or t
  misc_feature (26)..(29): n is a, c, g, or t
tgtaatacgactcactatagnnnnannnnggatccagcaggtagtgcgagg

SEQ ID NO: 89 - DNA, 51 bp, Artificial Sequence
  Synthetic Polynucleotide
  misc_feature (21)..(24): n is a, c, g, or t
  misc_feature (26)..(29): n is a, c, g, or t
tgtaatacgactcactatagnnnnannnncactgtgacatcggcccaaaag

SEQ ID NO: 90 - DNA, 51 bp, Artificial Sequence
  Synthetic Polynucleotide
  misc_feature (21)..(24): n is a, c, g, or t
  misc_feature (26)..(29): n is a, c, g, or t
tgtaatacgactcactatagnnnnannnnctgacagtgaccagtgcccatc

SEQ ID NO: 91 - DNA, 51 bp, Artificial Sequence
  Synthetic Polynucleotide
  misc_feature (21)..(24): n is a, c, g, or t
  misc_feature (26)..(29): n is a, c, g, or t
tgtaatacgactcactatagnnnnannnngagatccagtccacggagtcag

SEQ ID NO: 92 - DNA, 52 bp, Artificial Sequence
  Synthetic Polynucleotide
  misc_feature (21)..(24): n is a, c, g, or t
  misc_feature (26)..(29): n is a, c, g, or t
tgtaatacgactcactatagnnnnannnngtgaagttggcccacaccagcca

SEQ ID NO: 93 - DNA, 51 bp, Artificial Sequence
  Synthetic Polynucleotide
  misc_feature (21)..(24): n is a, c, g, or t
  misc_feature (26)..(29): n is a, c, g, or t
tgtaatacgactcactatagnnnnannnncctggcaatcctgtcctcagaa

SEQ ID NO: 94 - DNA, 51 bp, Artificial Sequence
  Synthetic Polynucleotide
  misc_feature (21)..(24): n is a, c, g, or t
  misc_feature (26)..(29): n is a, c, g, or t
tgtaatacgactcactatagnnnnannnngagtctgccatccccaaccaga

SEQ ID NO: 95 - DNA, 50 bp, Artificial Sequence
  Synthetic Polynucleotide
  misc_feature (21)..(24): n is a, c, g, or t
  misc_feature (26)..(29): n is a, c, g, or t
tgtaatacgactcactatagnnnnannnnggagtctgccaggccctcaca

SEQ ID NO: 96 - DNA, 51 bp, Artificial Sequence
  Synthetic Polynucleotide
  misc_feature (21)..(24): n is a, c, g, or t
  misc_feature (26)..(29): n is a, c, g, or t
tgtaatacgactcactatagnnnnannnngaagtctgccagcaccaaccag

SEQ ID NO: 97 - DNA, 51 bp, Artificial Sequence
  Synthetic Polynucleotide
  misc_feature (21)..(24): n is a, c, g, or t
  misc_feature (26)..(29): n is a, c, g, or t
tgtaatacgactcactatagnnnnannnnggagtcgcccagccccaaccag

SEQ ID NO: 98 - DNA, 51 bp, Artificial Sequence
  Synthetic Polynucleotide
  misc_feature (21)..(24): n is a, c, g, or t
  misc_feature (26)..(29): n is a, c, g, or t
tgtaatacgactcactatagnnnnannnnggagtccgccagcaccaaccag

SEQ ID NO: 99 - DNA, 52 bp, Artificial Sequence
  Synthetic Polynucleotide
  misc_feature (21)..(24): n is a, c, g, or t
  misc_feature (26)..(29): n is a, c, g, or t
tgtaatacgactcactatagnnnnannnngtgagcaacatgagccctgaaga

SEQ ID NO: 100 - DNA, 52 bp, Artificial Sequence
  Synthetic Polynucleotide
  misc_feature (21)..(24): n is a, c, g, or t
  misc_feature (26)..(29): n is a, c, g, or t
tgtaatacgactcactatagnnnnannnngagttctaagaagctccttctca

SEQ ID NO: 101 - DNA, 20 bp, Artificial Sequence
  Synthetic Polynucleotide
tgtaatacgactcactatag

SEQ ID NO: 102 - DNA, 25 bp, Artificial Sequence
  Synthetic Polynucleotide
ggccacagcactgttgctcttgaag

SEQ ID NO: 103 - DNA, 24 bp, Artificial Sequence
  Synthetic Polynucleotide
ccactgtgcacctccttcccattc

SEQ ID NO: 104 - DNA, 22 bp, Artificial Sequence
  Synthetic Polynucleotide
tcgaccagcttgacatcacagg

SEQ ID NO: 105 - DNA, 24 bp, Artificial Sequence
  Synthetic Polynucleotide
cagatttgttgctccaggccacag

SEQ ID NO: 106 - DNA, 23 bp, Artificial Sequence
  Synthetic Polynucleotide
tctgtgatatacacatcagaatc

SEQ ID NO: 107 - DNA, 24 bp, Artificial Sequence
  Synthetic Polynucleotide
gaatcaaaatcggtgaataggcag

SEQ ID NO: 108 - DNA, 24 bp, Artificial Sequence
  Synthetic Polynucleotide
ggcagacagacttgtcactggatt

SEQ ID NO: 109 - DNA, 22 bp, Artificial Sequence
  Synthetic Polynucleotide
taggacaccgaggtaaagccac

SEQ ID NO: 110 - DNA, 23 bp, Artificial Sequence
  Synthetic Polynucleotide
ctgggtgacgggtttggccctat

SEQ ID NO: 111 - DNA, 20 bp, Artificial Sequence
  Synthetic Polynucleotide
ttgacagcggaagtggttgc

SEQ ID NO: 112 - DNA, 25 bp, Artificial Sequence
  Synthetic Polynucleotide
ggctgctcaggcagtatctggagtc

SEQ ID NO: 113 - DNA, 25 bp, Artificial Sequence
  Synthetic Polynucleotide
gccaggcacaccagtgtggcctttt

SEQ ID NO: 114 - DNA, 78 bp, Artificial Sequence
  Synthetic Polynucleotide
aatgatacggcgaccaccgagatctacactctttccctacacgacgctcttccgatcttgtaatacgactcactatag

SEQ ID NO: 115 - DNA, 87 bp, Artificial Sequence
  Synthetic Polynucleotide
caagcagaagacggcatacgagatgcctaagtgactggagttcagacgtgtgctcttccgatcctcagctggtacacggcagggtca

SEQ ID NO: 116 - DNA, 88 bp, Artificial Sequence
  Synthetic Polynucleotide
caagcagaagacggcatacgagatgcctaagtgactggagttcagacgtgtgctcttccgatcaaacacagcgacctcgggtgggaac

SEQ ID NO: 117 - DNA, 326 bp, Artificial Sequence
  Synthetic Polynucleotide
atgtggggagctttccttctctatgtttccatgaagatgggaggcactgcaggacaaagccttgagcagccctctgaagtgacagctgtggaaggagccattgtccagataaactgcacgtaccagacatctgggttttatgggctgtcctggtaccagcaacatgatggcggagcacccacatttctttcttacaatgctctggatggtttggaggagacaggtcgtttttcttcattccttagtcgctctgatagttatggttacctccttctacaggagctccagatgaaagactctgcctcttacttctgcgctgtgagaga

SEQ ID NO: 118 - DNA, 326 bp, Artificial Sequence
  Synthetic Polynucleotide
atgtggggagttttccttctttatgtttccatgaagatgggaggcactacaggacaaaacattgaccagcccactgagatgacagctacggaaggtgccattgtccagatcaactgcacgtaccagacatctgggttcaacgggctgttctggtaccagcaacatgctggcgaagcacccacatttctgtcttacaatgttctggatggtttggaggagaaaggtcgtttttcttcattccttagtcggtctaaagggtacagttacctccttttgaaggagctccagatgaaagactctgcctcttacctctgtgctgtgagaga

SEQ ID NO: 119 - DNA, 338 bp, Artificial Sequence
  Synthetic Polynucleotide
atggctttgcagagcactctgggggcggtgtggctagggcttctcctcaactctctctggaaggttgcagaaagcaaggaccaagtgtttcagccttccacagtggcatcttcagagggagctgtggtggaaatcttctgtaatcactctgtgtccaatgcttacaacttcttctggtaccttcacttcccgggatgtgcaccaagactccttgttaaaggctcaaagccttctcagcagggacgatacaacatgacctatgaacggttctcttcatcgctgctcatcctccaggtgcgggaggcagatgctgctgtttactactgtgctgtggagga

SEQ ID NO: 120 - DNA, 343 bp, Artificial Sequence
  Synthetic Polynucleotide
atggcctctgcacccatctcgatgcttgcgatgctcttcacattgagtgggctgagagctcagtcagtggctcagccggaagatcaggtcaacgttgctgaagggaatcctctgactgtgaaatgcacctattcagtctctggaaacccttatcttttttggtatgttcaataccccaaccgaggcctccagttccttctgaaatacatcacaggggataacctggttaaaggcagctatggctttgaagctgaatttaacaagagccaaacctccttccacctgaagaaaccatctgcccttgtgagcgactccgctttgtacttctgtgctgtgagagaca

SEQ ID NO: 121 - DNA, 328 bp, Artificial Sequence
  Synthetic Polynucleotide
atgaggcaagtggcgagagtgatcgtgttcctgaccctgagtactttgagccttgctaagaccacccagcccatctccatggactcatatgaaggacaagaagtgaacataacctgtagccacaacaacattgctacaaatgattatatcacgtggtaccaacagtttcccagccaaggaccacgatttattattcaaggatacaagacaaaagttacaaacgaagtggcctccctgtttatccctgccgacagaaagtccagcactctgagcctgccccgggtttccctgagcgacactgctgtgtactactgcctcgtgggtgaca

SEQ ID NO: 122 - DNA, 340 bp, Artificial Sequence
  Synthetic Polynucleotide
atgaagacatttgctggattttcgttcctgtttttgtggctgcagctggactgtatgagtagaggagaggatgtggagcagagtcttttcctgagtgtccgagagggagacagctccgttataaactgcacttacacagacagctcctccacctacttatactggtataagcaagaacctggagcaggtctccagttgctgacgtatattttttcaaatatggacatgaaacaagaccaaagactcactgttctattgaataaaaaggataaacatctgtctctgcgcattgcagacacccagactggggactcagctatctacttctgtgcagagagta

SEQ ID NO: 123 - DNA, 340 bp, Artificial Sequence
  Synthetic Polynucleotide
atggagtcattcctgggaggtgttttgctgattttgtggcttcaagtggactgggtgaagagccaaaagatagaacagaattccgaggccctgaacattcaggagggtaaaacggccaccctgacctgcaactatacaaactattccccagcatacttacagtggtaccgacaagatccaggaagaggccctgttttcttgctactcatacgtgaaaatgagaaagaaaaaaggaaagaaagactgaaggtcacctttgataccacccttaaacagagtttgtttcatatcacagcctcccagcctgcagactcagctacctacctctgtgctctagaca

SEQ ID NO: 124 - DNA, 337 bp, Artificial Sequence
  Synthetic Polynucleotide
atggagaagatgcggagacctgtcctaattatattttgtctatgtcttggctgggcaaatggagaaaaccaggtggagcacagccctcattttctgggaccccagcagggagacgttgcctccatgagctgcacgtactctgtcagtcgttttaacaatttgcagtggtacaggcaaaatacagggatgggtcccaaacacctattatccatgtattcagctggatatgagaagcagaaaggaagactaaatgctacattactgaagaatggaagcagcttgtacattacagccgtgcagcctgaagattcagccacctatttctgtgctgtagatg

SEQ ID NO: 125 - DNA, 341 bp, Artificial Sequence
  Synthetic Polynucleotide
atgctcctgttgctcataccagtgctggggatgatttttgccctgagagatgccagagcccagtctgtgagccagcataaccaccacgtaattctctctgaagcagcctcactggagttgggatgcaactattcctatggtggaactgttaatctcttctggtatgtccagtaccctggtcaacaccttcagcttctcctcaagtacttttcaggggatccactggttaaaggcatcaagggctttgaggctgaatttataaagagtaaattctcctttaatctgaggaaaccctctgtgcagtggagtgacacagctgagtacttctgtgccgtgaatgc

SEQ ID NO: 126 - DNA, 341 bp, Artificial Sequence
  Synthetic Polynucleotide
atgctcctgctgctcgtcccagtgctcgaggtgatttttactctgggaggaaccagagcccagtcggtgacccagcttgacagccacgtctctgtctctgaaggaaccccggtgctgctgaggtgcaactactcatcttcttattcaccatctctcttctggtatgtgcaacaccccaacaaaggactccagcttctcctgaagtacacatcagcggccaccctggttaaaggcatcaacggttttgaggctgaatttaagaagagtgaaacctccttccacctgacgaaaccctcagcccatatgagcgacgcggctgagtacttctgtgttgtgagtga

SEQ ID NO: 127 - DNA, 341 bp, Artificial Sequence
  Synthetic Polynucleotide
atgctcctggagcttatcccactgctggggatacattttgtcctgagaactgccagagcccagtcagtgacccagcctgacatccacatcactgtctctgaaggagcctcactggagttgagatgtaactattcctatggggcaacaccttatctcttctggtatgtccagtcccccggccaaggcctccagctgctcctgaagtacttttcaggagacactctggttcaaggcattaaaggctttgaggctgaatttaagaggagtcaatcttccttcaatctgaggaaaccctctgtgcattggagtgatgctgctgagtacttctgtgctgtgggtgc

SEQ ID NO: 128 - DNA, 345 bp, Artificial Sequence
  Synthetic Polynucleotide
atgctcctgctgctcgtcccagtgctcgaggtgatttttaccctgggaggaaccagagcccagtcggtgacccagcttggcagccacgtctctgtctctgaaggagccctggttctgctgaggtgcaactactcatcgtctgttccaccatatctcttctggtatgtgcaataccccaaccaaggactccagcttctcctgaagtacacatcagcggccaccctggttaaaggcatcaacggttttgaggctgaatttaagaagagtgaaacctccttccacctgacgaaaccctcagcccatatgagcgacgcggctgagtacttctgtgctgtgagtgacaca

SEQ ID NO: 129 - DNA, 418 bp, Artificial Sequence
  Synthetic Polynucleotide
atgctcctggtgctcatcccactgctggggatacattttgtcctgagtgagaactgtcagagcccagtcagtgacccagcctgacatccgcatcactgtctctgaaggagcctcactggagttgagatgtaactattcctatggggcgatgttgtgggaagtcagggaccccaaacggagggaccggctgaagccatggcagaagaatgtggattgtgaagatttcatggacatttattagttccccaaattaatacttttataatttcttatgcctctctttactgcaatctctaaacataaattgtaaagatttcatggacacttatcacttccccaatcaatacccctgtgatttcctatgcctgtctttactttaatctcttaatcctgtcagctgaggaggatgtatgtcacc

SEQ ID NO: 130 - DNA, 341 bp, Artificial Sequence
  Synthetic Polynucleotide
atgctcctgctgctcgtcccagcgttccaggtgatttttaccctgggaggaaccagagcccagtctgtgacccagcttgacagccaagtccctgtctttgaagaagcccctgtggagctgaggtgcaactactcatcgtctgtttcagtgtatctcttctggtatgtgcaataccccaaccaaggactccagcttctcctgaagtatttatcaggatccaccctggttaaaggcatcaacggttttgaggctgaatttaacaagagtcaaacttccttccacttgaggaaaccctcagtccatataagcgacacggctgagtacttctgtgctgtgagtga

SEQ ID NO: 131 - DNA, 342 bp, Artificial Sequence
  Synthetic Polynucleotide
atgctcttagtggtcattctgctgcttggaatgttcttcacactgagaaccagaacccagtcggtgacccagcttgatggccacatcactgtctctgaagaagcccctctggaactgaagtgcaactattcctatagtggagttccttctctcttctggtatgtccaatactctagccaaagcctccagcttctcctcaaagacctaacagaggccacccaggttaaaggcatcagaggttttgaggctgaatttaagaagagcgaaacctccttctacctgaggaaaccatcaacccatgtgagtgatgctgctgagtacttctgtgctgtgggtgacagg

SEQ ID NO: 132 - DNA, 338 bp, Artificial Sequence
  Synthetic Polynucleotide
atgaattcttctccaggaccagcgattgcactattcttaatgtttgggggaatcaatggagattcagtggtccagacagaaggccaagtgctcccctctgaaggggattccctgattgtgaactgctcctatgaaaccacacagtacccttcccttttttggtatgtccaatatcctggagaaggtccacagctccacctgaaagccatgaaggccaatgacaagggaaggaacaaaggttttgaagccatgtaccgtaaagaaaccacttctttccacttggagaaagactcagttcaagagtcagactccgctgtgtacttctgtgctctgagtga

SEQ ID NO: 133 - DNA, 338 bp, Artificial Sequence
  Synthetic Polynucleotide
atgaactattctccaggcttagtatctctgatactcttactgcttggaagaacccgtggaaattcagtgacccagatggaagggccagtgactctctcagaagaggccttcctgactataaactgcacgtacacagccacaggatacccttcccttttctggtatgtccaatatcctggagaaggtctacagctcctcctgaaagccacgaaggctgatgacaagggaagcaacaaaggttttgaagccacataccgtaaagaaaccacttctttccacttggagaaaggctcagttcaagtgtcagactcagcggtgtacttctgtgctctgagtga

SEQ ID NO: 134 - DNA, 343 bp, Artificial Sequence
  Synthetic Polynucleotide
atgaaaaagcatctgacgaccttcttggtgattttgtggctttatttttatagggggaatggcaaaaaccaagtggagcagagtcctcagtccctgatcatcctggagggaaagaactgcactcttcaatgcaattatacagtgagccccttcagcaacttaaggtggtataagcaagatactgggagaggtcctgtttccctgacaatcatgactttcagtgagaacacaaagtcgaacggaagatatacagcaactctggatgcagacacaaagcaaagctctctgcacatcacagcctcccagctcagcgattcagcctcctacatctgtgtggtgagcg

SEQ ID NO: 135 - DNA, 340 bp, Artificial Sequence
  Synthetic Polynucleotide
acggagaagcccttgggagtttcattcttgatttcctcctggcagctgtgctgggtgaatagactacatacactggagcagagtccttcattcctgaatattcaggagggaatgcatgccgttcttaattgtacttatcaggagagaacactcttcaatttccactggttccggcaggatccggggagaagacttgtgtctttgaccttaattcaatcaagccagaaggagcagggagacaaatattttaaagaactgcttggaaaagaaaaattttatagtgtttggaatatcgcagcctctcatctgggagattcagccacctacttctgtgctttgc

SEQ ID NO: 136 - DNA, 337 bp, Artificial Sequence
  Synthetic Polynucleotide
atgatatccttgagagttttactggtgatcctgtggcttcagttaagctgggtttggagccaacggaaggaggtggagcaggatcctggacccttcaatgttccagagggagccactgtcgctttcaactgtacttacagcaacagtgcttctcagtctttcttctggtacagacaggattgcaggaaagaacctaagttgctgatgtccgtatactccagtggtaatgaagatggaaggtttacagcacagctcaatagagccagccagtatatttccctgctcatcagagactccaagctcagtgattcagccacctacctctgtgtggtgaaca

SEQ ID NO: 137 - DNA, 338 bp, Artificial Sequence
  Synthetic Polynucleotide
atgaaatccttgagagttttactagtgatcctgtggcttcagttgagctgggtttggagccaacagaaggaggtggagcagaattctggacccctcagtgttccagagggagccattgcctctctcaactgcacttacagtgaccgaggttcccagtccttcttctggtacagacaatattctgggaaaagccctgagttgataatgttcatatactccaatggtgacaaagaagatggaaggtttacagcacagctcaataaagccagccagtatgtttctctgctcatcagagactcccagcccagtgattcagccacctacctctgtgccgtgaa

SEQ ID NO: 138 - DNA, 345 bp, Artificial Sequence
  Synthetic Polynucleotide
atgaaatccttgagagttttactggtgatcctgtggcttcagttaagctgggtttggagccaacagaaggaggtggagcaggatcctggaccactcagtgttccagagggagccattgtttctctcaactgcacttacagcaacagtgcttttcaatacttcatgtggtacagacagtattccagaaaaggccctgagttgctgatgtacacatactccagtggtaacaaagaagatggaaggtttacagcacaggtcgataaatccagcaagtatatctccttgttcatcagagactcacagcccagtgattcagccacctacctctgtgcaatgagcgcacag

SEQ ID NO: 139 - DNA, 337 bp, Artificial Sequence
  Synthetic Polynucleotide
atgacatccattcgagctgtatttatattcctgtggctgcagctggacttggtgaatggagagaatgtggagcagcatccttcaaccctgagtgtccaggagggagacagcgctgttatcaagtgtacttattcagacagtgcctcaaactacttcccttggtataagcaagaacttggaaaaggacctcagcttattatagacattcgttcaaatgtgggcgaaaagaaagaccaacgaattgctgttacattgaacaagacagccaaacatttctccctgcacatcacagagacccaacctgaagactcggctgtctacttctgtgcagcaagta

SEQ ID NO: 140 - DNA, 340 bp, Artificial Sequence
  Synthetic Polynucleotide
atggcaggcattcgagctttatttatgtacttgtggctgcagctggactgggtgagcagaggagagagtgtggggctgcatcttcctaccctgagtgtccaggagggtgacaactctattatcaactgtgcttattcaaacagcgcctcagactacttcatttggtacaagcaagaatctggaaaaggtcctcaattcattatagacattcgttcaaatatggacaaaaggcaaggccaaagagtcaccgttttattgaataagacagtgaaacatctctctctgcaaattgcagctactcaacctggagactcagctgtctacttttgtgcagagaata

SEQ ID NO: 141 - DNA, 350 bp, Artificial Sequence
  Synthetic Polynucleotide
atgtcactttctagcctgctgaaggtggtcacagcttcactgtggctaggacctggcattgcccagaagataactcaaacccaaccaggaatgttcgtgcaggaaaaggaggctgtgactctggactgcacatatgacaccagtgatcaaagttatggtctattctggtacaagcagcccagcagtggggaaatgatttttcttatttatcaggggtcttatgacgagcaaaatgcaacagaaggtcgctactcattgaatttccagaaggcaagaaaatccgccaaccttgtcatctccgcttcacaactgggggactcagcaatgtatttctgtgcaatgagagaggg

SEQ ID NO: 142 - DNA, 344 bp, Artificial Sequence
  Synthetic Polynucleotide
atgtatacgtatgtaacaaacctgcgcgttgtgcacatgtaccctagaacgggtgaacagcctccatattctggagtagagtccttcattcattcctgagtatccgggagggaatgcacaacattcttaattgcacttatgaggagagaacgttctcttaacttctactggttctggcagggtctggaaaaggacttgtgtctttgaccttaattcaatcaagccagatggaggagggagacaaacattttaaagaagcgcttggaaaagagaagttttatagtgttttgaatatgctggtctctcatcctggagattcaggcacctacttctgtgctttgagg

SEQ ID NO: 143 - DNA, 329 bp, Artificial Sequence
  Synthetic Polynucleotide
atgaagcccaccctcatctcagtgcttgtgataatatttatactcagaggaacaagagcccagagagtgactcagcccgagaagctcctctctgtctttaaaggggccccagtggagctgaagtgcaactattcctattctgggagtcctgaactcttctggtatgtccagtactccagacaacgcctccagttactcttgagacacatctctagagagagcatcaaaggcttcactgctgaccttaacaaaggcgagacatctttccacctgaagaaaccatttgctcaagaggaagactcagccatgtattactgtgctctaagtgg

SEQ ID NO: 144 - DNA, 337 bp, Artificial Sequence
  Synthetic Polynucleotide
atggaaactctcctgggagtgtctttggtgattctatggcttcaactggctagggtgaacagtcaacagggagaagaggatcctcaggccttgagcatccaggagggtgaaaatgccaccatgaactgcagttacaaaactagtataaacaatttacagtggtatagacaaaattcaggtagaggccttgtccacctaattttaatacgttcaaatgaaagagagaaacacagtggaagattaagagtcacgcttgacacttccaagaaaagcagttccttgttgatcacggcttcccgggcagcagacactgcttcttacttctgtgctacggacg

SEQ ID NO: 145 - DNA, 333 bp, Artificial Sequence
  Synthetic Polynucleotide
atgctgtctgcttcctgctcaggacttgtgatcttgttgatattcagaaggaccagtggagactcggttacccagacagaaggcccagttaccctccctgagagggcagctctgacattaaactgcacttatcagtccagctattcaacttttctattctggtatgtccagtatctaaacaaagagcctgagctcctcctgaaaagttcagaaaaccaggagacggacagcagaggttttcaggccagtcctatcaagagtgacagttccttccacctggagaagccctcggtgcagctgtcggactctgccgtgtactactgcgctctgaga

SEQ ID NO: 146 - DNA, 350 bp, Artificial Sequence
  Synthetic Polynucleotide
atgctgactgccagcctgttgagggcagtcatagcctccatctgtgttgtatccagcatggctcagaaggtaactcaagcgcagactgaaatttctgtggtggagaaggaggatgtgaccttggactgtgtgtatgaaacccgtgatactacttattacttattctggtacaagcaaccaccaagtggagaattggttttccttattcgtcggaactcttttgatgagcaaaatgaaataagtggtcggtattcttggaacttccagaaatccaccagttccttcaacttcaccatcacagcctcacaagtcgtggactcagcagtatacttctgtgctctgagtgaggc

SEQ ID NO: 147 - DNA, 337 bp, Artificial Sequence
  Synthetic Polynucleotide
atggagaaaatgttggagtgtgcattcatagtcttgtggcttcagcttggctggttgagtggagaagaccaggtgacgcagagtcccgaggccctgagactccaggagggagagagtagcagtcttaactgcagttacacagtcagcggtttaagagggctgttctggtataggcaagatcctgggaaaggccctgaattcctcttcaccctgtattcagctggggaagaaaaggagaaagaaaggctaaaagccacattaacaaagaaggaaagctttctgcacatcacagcccctaaacctgaagactcagccacttatctctgtgctgtgcagg

SEQ ID NO: 148 - DNA, 336 bp, Artificial Sequence
  Synthetic Polynucleotide
atggagaccctcttgggcctgcttatcctttggctgcagctgcaatgggtgagcagcaaacaggaggtgacgcagattcctgcagctctgagtgtcccagaaggagaaaacttggttctcaactgcagtttcactgatagcgctatttacaacctccagtggtttaggcaggaccctgggaaaggtctcacatctctgttgcttattcagtcaagtcagagagagcaaacaagtggaagacttaatgcctcgctggataaatcatcaggacgtagtactttatacattgcagcttctcagcctggtgactcagccacctacctctgtgctgtgagg

SEQ ID NO: 149 - DNA, 331 bp, Artificial Sequence
  Synthetic Polynucleotide
atgaagaggatattgggagctctgctggggctcttgagtgcccaggtttgctgtgtgagaggaatacaagtggagcagagtcctccagacctgattctccaggagggagccaattccacgctgcggtgcaatttttctgactctgtgaacaatttgcagtggtttcatcaaaacccttggggacagctcatcaacctgttttacattccctcagggacaaaacagaatggaagattaagcgccacgactgtcgctacggaacgctacagcttattgtacatttcctcttcccagaccacagactcaggcgtttatttctgtgctgtggagc

SEQ ID NO: 150 - DNA, 364 bp, Artificial Sequence
  Synthetic Polynucleotide
atggacaagatcttaggagcatcatttttagttctgtggcttcaactatgctgggtgagtggccaacagaaggagaaaagtgaccagcagcaggtgaaacaaagtcctcaatctttgatagtccagaaaggagggatttcaattataaactgtgcttatgagaacactgcgtttgactactttccatggtaccaacaattccctgggaaaggccctgcattattgatagccatacgtccagatgtgagtgaaaagaaagaaggaagattcacaatctccttcaataaaagtgccaagcagttctcattgcatatcatggattcccagcctggagactcagccacctacttctgtgcagcaagca

SEQ ID NO: 151 - DNA, 343 bp, Artificial Sequence
  Synthetic Polynucleotide
atggagaagaatcctttggcagccccattactaatcctctggtttcatcttgactgcgtgagcagcatactgaacgtggaacaaagtcctcagtcactgcatgttcaggagggagacagcaccaatttcacctgcagcttcccttccagcaatttttatgccttacactggtacagatgggaaactgcaaaaagccccgaggccttgtttgtaatgactttaaatggggatgaaaagaagaaaggacgaataagtgccactcttaataccaaggagggttacagctatttgtacatcaaaggatcccagcctgaagactcagccacatacctctgtgccttta

SEQ ID NO: 152 - DNA, 327 bp, Artificial Sequence
  Synthetic Polynucleotide
atgctactcatcacatcaatgttggtcttatggatgcaattgtcacaggtgaatggacaacaggtaatgcaaattcctcagtaccagcatgtacaagaaggagaggacttcaccacgtactgcaattcctcaactactttaagcaatatacagtggtataagcaaaggcctggtggacatcccgtttttttgatacagttagtgaagagtggagaagtgaagaagcagaaaagactgacatttcagtttggagaagcaaaaaagaacagctccctgcacatcacagccacccagactacagatgtaggaacctacttctgtgcaggg

SEQ ID NO: 153 - DNA, 328 bp, Artificial Sequence
  Synthetic Polynucleotide
atgaggctggtggcaagagtaactgtgtttctgacctttggaactataattgatgctaagaccacccagcccccctccatggattgcgctgaaggaagagctgcaaacctgccttgtaatcactctaccatcagtggaaatgagtatgtgtattggtatcgacagattcactcccaggggccacagtatatcattcatggtctaaaaaacaatgaaaccaatgaaatggcctctctgatcatcacagaagacagaaagtccagcaccttgatcctgccccacgctacgctgagagacactgctgtgtactattgcatcgtcagagtcg

SEQ ID NO: 154 - DNA, 327 bp, Artificial Sequence
  Synthetic Polynucleotide
atgaagttggtgacaagcattactgtactcctatctttgggtattatgggtgatgctaagaccacacagccaaattcaatggagagtaacgaagaagagcctgttcacttgccttgtaaccactccacaatcagtggaactgattacatacattggtatcgacagcttccctcccagggtccagagtacgtgattcatggtcttacaagcaatgtgaacaacagaatggcctctctggcaatcgctgaagacagaaagtccagtaccttgatcctgcaccgtgctaccttgagagatgctgctgtgtactactgcatcctgagagac

SEQ ID NO: 155 - DNA, 328 bp, Artificial Sequence
  Synthetic Polynucleotide
atggtcctgaaattctccgtgtccattctttggattcagttggcatgggtgagcacccagctgctggagcagagccctcagtttctaagcatccaagagggagaaaatctcactgtgtactgcaactcctcaagtgttttttccagcttacaatggtacagacaggagcctggggaaggtcctgtcctcctggtgacagtagttacgggtggagaagtgaagaagctgaagagactaacctttcagtttggtgatgcaagaaaggacagttctctccacatcactgcagcccagcctggtgatacaggcctctacctctgtgcaggag

SEQ ID NO: 156 - DNA, 323 bp, Artificial Sequence
  Synthetic Polynucleotide
atgaaggcattaataggaatcttgctgggcttcctgtggatacagatttgctcgcaaatgaaagtggagcagagtcctcaggtcctgatcctccaagagggaagaaattcattcctggtgtgcagttgttctatttacatgatccgtgtgcagtggtttcatcaaaagcctggaggacccctcatgtccttatttaacattaattcaggaatacagcaaaaaagaagactaaaatccgcagtcaaagctgaggaactttatggccacctatacatcagattcccagcctgaggactcagctatttacttctgtgctgtgggga

SEQ ID NO: 157 - DNA, 358 bp, Artificial Sequence
  Synthetic Polynucleotide
atggccatgctcctgggggcatcagtgctgattctgtggcttcagccagactgggtaaacagtcaacagaagaatgatgaccagcaagttaagcaaaattcaccatccctgagcgtccaggaaggaagaatttctattctgaactgtgactatactaacagcatgtttgattatttcctatggtacaaaaaataccctgctgaaggtcctacattcctgatatctataagttccattaaggataaaaatgaagatggaagattcactgtcttcttaaacaaaagtgccaagcacctctctctgcacattgtgccctcccagcctggagactctgcagtgtacttctgtgcagcaagcg

SEQ ID NO: 158 - DNA, 337 bp, Artificial Sequence
  Synthetic Polynucleotide
atggagactctcctgaaagtgctttcaggcaccttgttgtggcagttgacctgggtgagaagccaacaaccagtgcagagtcctcaagccgtgatcctccgagaaggggaagatgctgtcatcaactgcagttcctccaaggctttatattctgtacactggtacaggcagaagcatggtgaagcacccgtcttcctgatgatattactgaagggtggagaacagaagggtcatgaaaaaatatctgcttcatttaatgaaaaaaagcagcaaagctccctgtaccttacggcctcccagctcagttactcaggaacctacttctgcggcacagaga

SEQ ID NO: 159 - DNA, 342 bp, Artificial Sequence
  Synthetic Polynucleotide
atgactgttggcagcatattacgggcactcatggcctctgccttccttgcatgtcacagagggtcattcaatcccaaccagcaatatctacgcaggagggtgagaccgtgaaactggactgtgcatacaaaactaatattgtatattacatattgtattggtacaaaaggtctcccaatgggaagattattttcctcatttatcagcaaacagatgcagaaaccaatgcgacacagggtcaatattctgtgagcttccagaaaacaactaaaactattcagcttatcatatcatcatcacagccagaagacctgcaacatatttctgttgtctcaaagagcc

SEQ ID NO: 160 - DNA, 344 bp, Artificial Sequence
  Synthetic Polynucleotide
atggcaagaagaatggaaaagtccctgggagctttattcaaattcagctgaagctggccaagaaaaggatgtgatacagagttattcaaatctaaatgtctaggagagagaaatggccgttattaatgacagttatacagatggagctttgaattatttctgttggtacaagaagaaaacggggaaggccctaatatcttaatggagattcattcaaatgtggatagaaaacaggacagaaggctcactgtactgttgaataaaaatgctaaacatgtctccctgcatattacagccacccaaccaggagactcattcctgtacttctgtgcagtgagaacaca

SEQ ID NO: 161 - DNA, 338 bp, Artificial Sequence
  Synthetic Polynucleotide
atgctctgccctggcctgctgtgggcattcgtggtcccctttggcttcagatccagcatggctcagaaagtaacccaagttcagaccacagtaactaggcagaaaggagtagctgtgaccttggactgcatgtttgaaaccagatagaattcgtacactttatactggtacaagcaacaagcaacctcccagtgaagagatggttttccttattcatcagggttattctaagtcaaatgcaaagcctgtgaactttgaaaaaaagaaaaagttcatcaacctcaccatcaattccttaaaactgactcagccaagtacttctgtgctctcaggaatcc

SEQ ID NO: 162 - DNA, 337 bp, Artificial Sequence
  Synthetic Polynucleotide
atggagactgttctgcaagtactcctagggatattggggttccaagcagcctgggtcagtagccaagaactggagcagagtcctcagtccttgatcgtccaagagggaaagaatctcaccataaactgcacgtcatcaaagacgttatatggcttatactggtataagcaaaagtatggtgaaggtcttatcttcttgatgatgctacagaaaggtggggaagagaaaagtcatgaaaagataactgccaagttggatgagaaaaagcagcaaagttccctgcatatcacagcctcccagcccagccatgcaggcatctacctctgtggagcagaca

SEQ ID NO: 163 - DNA, 330 bp, Artificial Sequence
  Synthetic Polynucleotide
atgctccttgaacatttattaataatcttgtggatgcagctgacatgggtcagtggtcaacagctgaatcagagtcctcaatctatgtttatccaggaaggagaagatgtctccatgaactgcacttcttcaagcatatttaacacctggctatggtacaagcaggaacctggggaaggtcctgtcctcttgatagccttatataaggctggtgaattgacctcaaatggaagactgactgctcagtttggtataaccagaaaggacagcttcctgaatatctcagcatccatacctagtgatgtaggcatctacttctgtgctgggcag

SEQ ID NO: 164 - DNA, 340 bp, Artificial Sequence
  Synthetic Polynucleotide
atgatgaagtgtccacaggctttactagctatcttttggcttctactgagctgggtgagcagtgaagacaaggtggtacaaagccctctatctctggttgtccacgagggagacaccgtaactctcaattgcagttatgaagtgactaactttcgaagcctactatggtacaagcaggaaaagaaagctcccacatttctatttatgctaacttcaagtggaattgaaaagaagtcaggaagactaagtagcatattagataagaaagaactttccagcatcctgaacatcacagccacccagaccggagactcggccatctacctctgtgctgtggagg

SEQ ID NO: 165 - DNA, 342 bp, Artificial Sequence
  Synthetic Polynucleotide
atggaaactccactgagcactctgctgctgctcctctgtgtgcagctgacctggtcaaatggacaactgccagtggaacagaatgctccttccctgaaagtcaaggaaggtgacagcgtcacactgaactgcagttacagagacagcccttcagatttcttcagtggttcaggcaggatcctgaggaaggcctcatttccctgatacaaatgctatcaactgtgagagagaagatcagtggaagattcacagccaggcttaaaaaaggagaccagcacatttccctgcacatacaggattcccagctccatgactcaaccacattcttctgcgcagcaagca

SEQ ID NO: 166 - DNA, 350 bp, Artificial Sequence
  Synthetic Polynucleotide
atgacacgagttagcttgctgtgggcagtcgtggtctccacctgtcttgaatccggcatggcccagacagtcactcagtctcaaccagagatgtctgtgcaggaggcagagactgtgaccctgagttgcacatatgacaccagtgagaataattattatttgttctggtacaagcagcctcccagcaggcagatgattctcgttattcgccaagaagcttataagcaacagaatgcaacggagaatcgtttctctgtgaacttccagaaagcagccaaatccttcagtctcaagatctcagactcacagctgggggacactgcgatgtatttctgtgctttcatgaagca

SEQ ID NO: 167 - DNA, 349 bp, Artificial Sequence
  Synthetic Polynucleotide
atggcatgccctggcttcctgtgggcacttgtgatctccacctgtcttgaatttagcatggctcagacagtcactcagtctcaaccagagatgtctgtgcaggaggcagagaccgtgaccctgagctgcacatatgacaccagtgagagtgattattatttattctggtacaagcagcctcccagcaggcagatgattctcgttattcgccaagaagcttataagcaacagaatgcaacagagaatcgtttctctgtgaacttccagaaagcagccaaatccttcagtctcaagatctcagactcacagctgggggatgccgcgatgtatttctgtgcttataggagcg

SEQ ID NO: 168 - DNA, 331 bp, Artificial Sequence
  Synthetic Polynucleotide
atgaagaagctactagcaatgattctgtggcttcaactagaccggttaagtggagagctgaaagtggaacaaaaccctctgttcctgagcatgcaggagggaaaaaactataccatctactgcaattattcaaccacttcagacagactgtattggtacaggcaggatcctgggaaaagtctggaatctctgtttgtgttgctatcaaatggagcagtgaagcaggagggacgattaatggcctcacttgataccaaagcccgtctcagcaccctccacatcacagctgccgtgcatgacctctctgccacctacttctgtgccgtggaca

SEQ ID NO: 169 - DNA, 317 bp, Artificial Sequence
  Synthetic Polynucleotide
atgaactcctctctggactttctaattctgatcttaatgtttggaggaaccagcagcaattcagtcaagcagacgggccaaataaccgtctcggagggagcatctgtgactatgaactgcacatacacatccacggggtaccctacccttttctggtatgtggaataccccagcaaacctctgcagcttcttcagagagagacaatggaaaacagcaaaaacttcggaggcggaaatattaaagacaaaaactcccccattgtgaaatattcagtccaggtatcagactcagccgtgtactactgtcttctgggaga

SEQ ID NO: 170 - DNA, 336 bp, Artificial Sequence
  Synthetic Polynucleotide
atggtgaagatccggcaatttttgttggctattttgtggcttcagctaagctgtgtaagtgccgccaaaaatgaagtggagcagagtcctcagaacctgactgcccaggaaggagaatttatcacaatcaactgcagttactcggtaggaataagtgccttacactggctgcaacagcatccaggaggaggcattgtttccttgtttatgctgagctcagggaagaagaagcatggaagattaattgccacaataaacatacaggaaaagcacagctccctgcacatcacagcctcccatcccagagactctgccgtctacatctgtgctgtcaga

SEQ ID NO: 171 - DNA, 333 bp, Artificial Sequence
  Synthetic Polynucleotide
atgggctgaagtctccactgtggtgtggtccattgtctcaggctccatggatactggaattacccagacaccaaaatacctggtcacagcaatggggagtaaaaggacaatgaaacgtgagcatctgggacatgattctatgtattggtacagacagaaagctaagaaatccctggagttcatgttttactacaactgtaaggaattcattgaaaacaagactgtgccaaatcacttcacacctgaatgccctgacagctctcgcttataccttcatgtggtcgcactgcagcaagaagactcagctgcgtatctctgcaccagcagccaaga

SEQ ID NO: 172 - DNA, 347 bp, Artificial Sequence
  Synthetic Polynucleotide
atggatacctggctcgtatgctgggcaatttttagtctcttgaaagcaggactcacagaacctgaagtcacccagactcccagccatcaggtcacacagatgggacaggaagtgatcttgcgctgtgtccccatctctaatcacttatacttctattggtacagacaaatcttggggcagaaagtcgagtttctggtttccttttataataatgaaatctcagagaagtctgaaatattcgatgatcaattctcagttgaaaggcctgatggatcaaatttcactctgaagatccggtccacaaagctggaggactcagccatgtacttctgtgccagcagtgaagc

SEQ ID NO: 173 - DNA, 344 bp, Artificial Sequence
  Synthetic Polynucleotide
atgggctgcaggctcctctgctgtgtggtcttctgcctcctccaagcaggtcccttggacacagctgtttcccagactccaaaatacctggtcacacagatgggaaacgacaagtccattaaatgtgaacaaaatctgggccatgatactatgtattggtataaacaggactctaagaaatttctgaagataatgtttagctacaataataaggagctcattataaatgaaacagttccaaatcgcttctcacctaaatctccagacaaagctcacttaaatcttcacatcaattccctggagcttggtgactctgctgtgtatttctgtgccagcagccaaga

SEQ ID NO: 174 - DNA, 345 bp, Artificial Sequence
  Synthetic Polynucleotide
atgggctgcaggctcctctgctatgtggccctctgcctcctgcaagcaggatccactggacacagccgtttcccagactccaaaatacctggtcacacagatgggaaaaaaggagtctcttaaatgagaacaaaatctgggccataatgctatgtattggtataaacaggactctaagaaatttctgaagacaatgtttatctacagtaacaaggagccaattttaaatgaaacagttccaaatcgcttctcacctgactctccagacaaagctcatttaaatcttcacatcaattccctggagcttggtgactctgctgtgtatttctgtgccagcagccaaga

SEQ ID NO: 175 - DNA, 344 bp, Artificial Sequence
  Synthetic Polynucleotide
atgggctgcaggctgctctgctgtgcggttctctgtctcctgggagcagttcccatagacactgaagttacccagacaccaaaacacctggtcatgggaatgacaaataagaagtctttgaaatgtgaacaacatatggggcacagggctatgtattggtacaagcagaaagctaagaagccaccggagctcatgtttgtctacagctatgagaaactctctataaatgaaagtgtgccaagtcgcttctcacctgaatgccccaacagctctctcttaaaccttcacctacacgccctgcagccagaagactcagccctgtatctctgcgccagcagccaaga

SEQ ID NO: 176 - DNA, 344 bp, Artificial Sequence
  Synthetic Polynucleotide
atgggctgcaggctgctctgctgtgcggttctctgtctcctgggagcggtccccatggaaacgggagttacgcagacaccaagacacctggtcatgggaatgacaaataagaagtctttgaaatgtgaacaacatctggggcataacgctatgtattggtacaagcaaagtgctaagaagccactggagctcatgtttgtctacaactttaaagaacagactgaaaacaacagtgtgccaagtcgcttctcacctgaatgccccaacagctctcacttattccttcacctacacaccctgcagccagaagactcggccctgtatctctgtgccagcagccaaga

SEQ ID NO: 177 - DNA, 353 bp, Artificial Sequence
  Synthetic Polynucleotide
atgggctgcaggctgctctgctgtgcggttctctgtctcctgggagcgggtgagttggtccccatggaaacgggagttacgcagacaccaagacacctggtcatgggaatgacaaataagaagtctttgaaatgtgaacaacatctgggtcataacgctatgtattggtacaagcaaagtgctaagaagccactggagctcatgtttgtctacagtcttgaagaacgggttgaaaacaacagtgtgccaagtcgcttctcacctgaatgccccaacagctctcacttattccttcacctacacaccctgcagccagaagactcggccctgtatctctgcgccagcagccaaga

SEQ ID NO: 178 - DNA, 343 bp, Artificial Sequence
  Synthetic Polynucleotide
atgggctccaggctgctctgttgggtgctgctttgtctcctgggagcaggcccagtaaaggctggagtcactcaaactccaagatatctgatcaaaacgagaggacagcaagtgacactgagctgctcccctatctctgggcataggagtgtatcctggtaccaacagaccccaggacagggccttcagttcctctttgaatacttcagtgagacacagagaaacaaaggaaacttccctggtcgattctcagggcgccagttctctaactctcgctctgagatgaatgtgagcaccttggagctgggggactcggccctttatctttgcgccagcagcttgg

SEQ ID NO: 179 - DNA, 331 bp, Artificial Sequence
  Synthetic Polynucleotide
atgggctccggactcctctgctggacgctgctttgtttcctgggagcaggcccagtggaggctggaatcacccaagctccaagacacctgatcaaaacaagagaccagcaagtgacactgagatgctcccctgcctctgggcataactgtgtgtcctggtacctacgaactccaagtcagcccctctagttattgttacaatattgtaataggttacaaagagcaaaaggaaacttgcctaattgattctcagctcaccacgtccataactattactgagtcaaacacggagctaggggactcagccctgtatctctgtgccagcaacttg

SEQ ID NO: 180 - DNA, 343 bp, Artificial Sequence
  Synthetic Polynucleotide
atgggccccgggctcctctgctgggaactgctttatctcctgggagcaggcccagtggaggctggagtcacccaaagtcccacacacctgatcaaaacgagaggacagcaagtgactctgagatgctctcctatctctgggcacagcagtgtgtcctggtaccaacaggccccgggtcaggggccccagtttatctttgaatatgctaatgagttaaggagatcagaaggaaacttccctaatcgattctcagggcgccagttccatgactgttgctctgagatgaatgtgagtgccttggagctgggggactcggccctgtatctctgtgccagaagcttgg

SEQ ID NO: 181 - DNA, 343 bp, Artificial Sequence
  Synthetic Polynucleotide
atgggccctgggctcctctgctgggtgctgctttgtctcctgggagcaggctcagtggagactggagtcacccaaagtcccacacacctgatcaaaacgagaggacagcaagtgactctgagatgctcttctcagtctgggcacaacactgtgtcctggtaccaacaggccctgggtcaggggccccagtttatctttcagtattatagggaggaagagaatggcagaggaaacttccctcctagattctcaggtctccagttccctaattatagctctgagctgaatgtgaacgccttggagctggacgactcggccctgtatctctgtgccagcagcttgg

SEQ ID NO: 182 - DNA, 343 bp, Artificial Sequence
  Synthetic Polynucleotide
atgggccctgggctcctctgctgggtgctgctttgtctcctgggagcaggcccagtggacgctggagtcacccaaagtcccacacacctgatcaaaacgagaggacagcaagtgactctgagatgctctcctatctctgggcacaagagtgtgtcctggtaccaacaggtcctgggtcaggggccccagtttatctttcagtattatgagaaagaagagagaggaagaggaaacttccctgatcgattctcagctcgccagttccctaactatagctctgagctgaatgtgaacgccttgttgctgggggactcggccctgtatctctgtgccagcagcttgg

SEQ ID NO: 183 - DNA, 343 bp, Artificial Sequence
  Synthetic Polynucleotide
atgggccccgggctcctctgctgggcactgctttgtctcctgggagcaggcttagtggacgctggagtcacccaaagtcccacacacctgatcaaaacgagaggacagcaagtgactctgagatgctctcctaagtctgggcatgacactgtgtcctggtaccaacaggccctgggtcaggggccccagtttatctttcagtattatgaggaggaagagagacagagaggcaacttccctgatcgattctcaggtcaccagttccctaactatagctctgagctgaatgtgaacgccttgttgctgggggactcggccctctatctctgtgccagcagcttgg

SEQ ID NO: 184 - DNA, 343 bp, Artificial Sequence
  Synthetic Polynucleotide
atgggccccgggctcctctgctgggtgctgctttgtcccctaggagaaggcccagtggacgctggagtcacccaaagtcccacacacctgatcaaaacgagaggacagcacgtgactctgagatgctctcctatctctgggcacaccagtgtgtcctcgtaccaacaggccctgggtcaggggccccagtttatctttcagtattatgagaaagaagagagaggaagaggaaacttccctgatcaattctcaggtcaccagttccctaactatagctctgagctgaatgtgaacgccttgttgctaggggactcggccctctatctctgtgccagcagcttgg

SEQ ID NO: 185 - DNA, 343 bp, Artificial Sequence
  Synthetic Polynucleotide
atgggacccaggctcctcttctgggcactgctttgtctcctcggaacaggcccagtggaggctggagtcacacaaagtcccacacacctgatcaaaacgagaggacagcaagcgactctgagatgctctcctatctctgggcacaccagtgtgtactggtaccaacaggccctgggtctgggcctccagttcctcctttggtatgacgagggtgaagagagaaacagaggaaacttccctcctagattttcaggtcgccagttccctaattatagctctgagctgaatgtgaacgccttggagctggaggactcggccctgtatctctgtgccagcagcttgg

SEQ ID NO: 186 - DNA, 344 bp, Artificial Sequence
  Synthetic Polynucleotide
atgagcatcgggctcctgtgctgtgtggccttttctctcctgtgggcaagtccagtgaatgctggtgtcactcagaccccaaaattccaggtcctgaagacaggacagagcatgacactgcagtgtgcccaggatatgaaccataactccatgtactggtatcgacaagacccaggcatgggactgaggctgatttattactcagcttctgagggtaccactgacaaaggagaagtccccaatggctacaatgtctccagattaaacaaacgggagttctcgctcaggctggagtcggctgctccctcccagacatctgtgtacttctgtgccagcagtgaagc

SEQ ID NO: 187 - DNA, 344 bp, Artificial Sequence
  Synthetic Polynucleotide
atgagcctcgggctcctgtgctgtggggccttttctctcctgtgggcaggtccagtgaatgctggtgtcactcagaccccaaaattccgggtcctgaagacaggacagagcatgacactgctgtgtgcccaggatatgaaccatgaatacatgtactggtatcgacaagacccaggcatggggctgaggctgattcattactcagttggtgagggtacaactgccaaaggagaggtccctgatggctacaatgtctccagattaaaaaaacagaatttcctgctggggttggagtcggctgctccctcccaaacatctgtgtacttctgtgccagcagttactc

SEQ ID NO: 188 - DNA, 344 bp, Artificial Sequence; identical to SEQ ID NO: 187
  Synthetic Polynucleotide

SEQ ID NO: 189 - DNA, 344 bp, Artificial Sequence
  Synthetic Polynucleotide
atgagaatcaggctcctgtgctgtgtggccttttctctcctgtgggcaggtccagtgattgctgggatcacccaggcaccaacatctcagatcctggcagcaggacggcgcatgacactgagatgtacccaggatatgagacataatgccatgtactggtatagacaagatctaggactggggctaaggctcatccattattcaaatactgcaggtaccactggcaaaggagaagtccctgatggttatagtgtctccagagcaaacacagatgatttccccctcacgttggcgtctgctgtaccctctcagacatctgtgtacttctgtgccagcagtgactc

SEQ ID NO: 190 - DNA, 344 bp, Artificial Sequence
  Synthetic Polynucleotide
atgagcatcggcctcctgtgctgtgcagccttgtctctcctgtgggcaggtccagtgaatgctggtgtcactcagaccccaaaattccaggtcctgaagacaggacagagcatgacactgcagtgtgcccaggatatgaaccatgaatacatgtcctggtatcgacaagacccaggcatggggctgaggctgattcattactcagttggtgctggtatcactgaccaaggagaagtccccaatggctacaatgtctccagatcaaccacagaggatttcccgctcaggctgctgtcggctgctccctcccagacatctgtgtacttctgtgccagcagttactc

SEQ ID NO: 191 - DNA, 344 bp, Artificial Sequence
  Synthetic Polynucleotide
atgagcatcagcctcctgtgctgtgcagcctttcctctcctgtgggcaggtccagtgaatgctggtgtcactcagaccccaaaattccgcatcctgaagataggacagagcatgacactgcagtgtacccaggatatgaaccataactacatgtactggtatcgacaagacccaggcatggggctgaagctgatttattattcagttggtgctggtatcactgataaaggagaagtcccgaatggctacaacgtctccagatcaaccacagaggatttcccgctcaggctggagttggctgctccctcccagacatctgtgtacttctgtgccagcagttactc

SEQ ID NO: 192 - DNA, 344 bp, Artificial Sequence
  Synthetic Polynucleotide
atgagcctcgggctcctgtgctgtgtggccttttctctcctgtgggcaggtccaatgaatgctggtgtcactcagaccccaaaattccacgtcctgaagacaggacagagcatgactctgctgtgtgcccaggatatgaaccatgaatacatgtatcggtatcgacaagacccaggcaaggggctgaggctgatttactactcagttgctgctgctctcactgacaaaggagaagttcccaatggctacaatgtctccagatcaaacacagaggatttccccctcaagctggagtcagctgctccctctcagacttctgtttacttctgtgccagcagttactc

SEQ ID NO: 193 - DNA, 341 bp, Artificial Sequence
  Synthetic Polynucleotide
atgagcctcgggctcctgtgctgtgcggccttttctctcctgtgggcaggtcccgtgaatgctggtgtcactcagaccccaaaattccacatcctgaagacaggacagagcatgacactgcagtgtgcccaggatatgaaccatggatacatgtcctggtatcgacaagacccaggcatggggctgagactgatttactactcagctgctgctggtactactgacaaagaagtccccaatggctacaatgtctctagattaaacacagaggatttcccactcaggctggtgtcggctgctccctcccagacatctgtgtacttgtgtgccagcagttactc

SEQ ID NO: 194 - DNA, 344 bp, Artificial Sequence
  Synthetic Polynucleotide
atgagcatcgggctcctgtgctgtgtggccttttctctcctgtgggagggtccagtgaatgctggtgtcactcagaccccaaaattccacatcctgaagacaggacagagcatgacactgcagtgtgcccaggatatgaaccatggatacttgtcctggtatcgacaagacccaggcatggggctgaggcgcattcattactcagttgctgctggtatcactgacaaaggagaagtccccgatggctacaatgtatccagatcaaacacagaggatttcccgctcaggctggagtcagctgctccctcccagacatctgtatacttctgtgccagcagttattc

SEQ ID NO: 195 - DNA, 347 bp, Artificial Sequence
  Synthetic Polynucleotide
atgggcacaaggctcctctgctgggcagccatatgtctcctgggggcagatcacacaggtgctggagtctcccagtccctgagacacaaggtagcaaagaagggaaaggatgtagctctcagatatgatccaatttcaggtcataatgccctttattggtaccgacagagcctggggcagggcctggagtttccaatttacttccaaggcaaggatgcagcagacaaatcggggcttccccgtgatcggttctctgcacagaggtctgagggatccatctccactctgaagttccagcgcacacagcagggggacttggctgtgtatctctgtgccagcagctcagc

SEQ ID NO: 196 - DNA, 347 bp, Artificial Sequence
  Synthetic Polynucleotide
atgggcaccaggctcctcttctgggtggccttctgtctcctgggggcagatcacacaggagctggagtctcccagtcccccagtaacaaggtcacagagaagggaaaggatgtagagctcaggtgtgatccaatttcaggtcatactgccctttactggtaccgacagagcctggggcagggcctggagtttttaatttacttccaaggcaacagtgcaccagacaaatcagggctgcccagtgatcgcttctctgcagagaggactgggggatccgtctccactctgacgatccagcgcacacagcaggaggactcggccgtgtatctctgtgccagcagcttagc

SEQ ID NO: 197 - DNA, 347 bp, Artificial Sequence
  Synthetic Polynucleotide
atgggcaccaggctcctctgctgggcagccctgtgcctcctgggggcagatcacacaggtgctggagtctcccagacccccagtaacaaggtcacagagaagggaaaatatgtagagctcaggtgtgatccaatttcaggtcatactgccctttactggtaccgacaaagcctggggcagggcccagagtttctaatttacttccaaggcacgggtgcggcagatgactcagggctgcccaacgatcggttctttgcagtcaggcctgagggatccgtctctactctgaagatccagcgcacagagcggggggactcagccgtgtatctctgtgccagcagcttaac

SEQ ID NO: 198 - DNA, 347 bp, Artificial Sequence
  Synthetic Polynucleotide
atgggcaccaggctcctctgctgggtggtcctgggtttcctagggacagatcacacaggtgctggagtctcccagtccccaaggtacaaagtcgcaaagaggggacgggatgtagctctcaggtgtgattcaatttcgggtcatgtaaccctttattggtaccgacagaccctggggcagggctcagaggttctgacttactcccagagtgatgctcaacgagacaaatcagggcggcccagtggtcggttctctgcagagaggcctgagagatccgtctccactctgaagatccagcgcacagagcagggggactcagctgtgtatctctgtgccagcagcttagc

SEQ ID NO: 199 - DNA, 345 bp, Artificial Sequence
  Synthetic Polynucleotide
atgggcaccaggctcctctgctgggtggtcctgggtttcctagggacagatcacacaggtgctggagtctcccagtccccaaggtacgaagtcacacagaggggacaggatgtagctcccaggtgtgatccaatttcgggtcaggtaaccctttattggtaccgacagaccctggggcagggccaagagtttctgacttccttccaggatgaaactcaacaagataaatcagggctgctcagtgatcaattctccacagagaggtctgaggatctttctccacctgaagatccagcgcacagagcaagggcgactcggctgtgtatctctgtgccagaagcttag

SEQ ID NO: 200 - DNA, 347 bp, Artificial Sequence
  Synthetic Polynucleotide
atgggcaccagtctcctatgctgggtggtcctgggtttcctagggacagatcacacaggtgctggagtctcccagtctcccaggtacaaagtcacaaagaggggacaggatgtagctctcaggtgtgatccaatttcgggtcatgtatccctttattggtaccgacaggccctggggcagggcccagagtttctgacttacttcaattatgaagcccaacaagacaaatcagggctgcccaatgatcggttctctgcagagaggcctgagggatccatctccactctgacgatccagcgcacagagcagcgggactcggccatgtatcgctgtgccagcagcttagc

SEQ ID NO: 201 - DNA, 347 bp, Artificial Sequence
  Synthetic Polynucleotide
atgggtaccagtctcctatgctgggtggtcctgggtttcctagggacagatcacacaggtgctggagtctcccagtctcccaggtacaaagtcacaaagaggggacaggatgtaactctcaggtgtgatccaatttcgagtcatgcaaccctttattggtatcaacaggccctggggcagggcccagagtttctgacttacttcaattatgaagctcaaccagacaaatcagggctgcccagtgatcggttctctgcagagaggcctgagggatccatctccactctgacgattcagcgcacagagcagcgggactcagccatgtatcgctgtgccagcagcttagc

SEQ ID NO: 202 - DNA, 347 bp, Artificial Sequence
  Synthetic Polynucleotide
atgggcaccaggctcctctgctgggtggtcctgggtttcctagggacagatcacacaggtgctggagtctcccagtcccctaggtacaaagtcgcaaagagaggacaggatgtagctctcaggtgtgatccaatttcgggtcatgtatcccttttttggtaccaacaggccctggggcaggggccagagtttctgacttatttccagaatgaagctcaactagacaaatcggggctgcccagtgatcgcttctttgcagaaaggcctgagggatccgtctccactctgaagatccagcgcacacagcaggaggactccgccgtgtatctctgtgccagcagcttagc

SEQ ID NO: 203 - DNA, 347 bp, Artificial Sequence
  Synthetic Polynucleotide
atgggcaccagcctcctctgctggatggccctgtgtctcctgggggcagatcacgcagatactggagtctcccagaaccccagacacaagatcacaaagaggggacagaatgtaactttcaggtgtgatccaatttctgaacacaaccgcctttattggtaccgacagaccctggggcagggcccagagtttctgacttacttccagaatgaagctcaactagaaaaatcaaggctgctcagtgatcggttctctgcagagaggcctaagggatctttctccaccttggagatccagcgcacagagcagggggactcggccatgtatctctgtgccagcagcttagc

SEQ ID NO: 204 - DNA, 279 bp, Artificial Sequence
  Synthetic Polynucleotide
gaggcagggatcagccagataccaagatatcacagacacacagggaaaaagatcatcctgaaatatgctcagattaggaaccattattcagtgttctgttatcaataagaccaagaataggggctgaggctgatccattattcaggtagtattggcagcatgaccaaaggcggtgccaaggaagggtacaatgtctctggaaacaagctcaagcattttccctcaaccctggagtctactagcaccagccagacctctgtacctctgtggcagtgcatc

SEQ ID NO: 205 - DNA, 325 bp, Artificial Sequence
  Synthetic Polynucleotide
atgaaccccaaactcttctgtgtgaccctttgtctcctgggagcaggctctattgatgctgggatcacccagatgccaagatatcacattgtacagaagaaagagatgatcctggaatgtgctcaggttaggaacagtgttctgatatcgacaggacccaagacgggggctgaagcttatccactattcaggcagtggtcacagcaggaccaaagttgatgtcacagaggggtactgtgtttcttgaaacaagcttgagcatttccccaatcctggcatccaccagcaccagccagacctatctgtaccactgtggcagcacatc

SEQ ID NO: 206 - DNA, 343 bp, Artificial Sequence
  Synthetic Polynucleotide
atgggcttcaggctcctctgctgtgtggccttttgtctcctgggagcaggcccagtggattctggagtcacacaaaccccaaagcacctgatcacagcaactggacagcgagtgacgctgagatgctcccctaggtctggagacctctctgtgtactggtaccaacagagcctggaccagggcctccagttcctcattcagtattataatggagaagagagagcaaaaggaaacattcttgaacgattctccgcacaacagttccctgacttgcactctgaactaaacctgagctctctggagctgggggactcagctttgtatttctgtgccagcagcgtag

SEQ ID NO: 207 - DNA, 344 bp, Artificial Sequence
  Synthetic Polynucleotide
atgggcacgaggctcttcttctatgtggccctttgtctgctgtgggcaggacacagggatgctgaaatcacccagagcccaagacacaagatcacagagacaggaaggcaggtgaccttggcgtgtcaccagacttggaaccacaacaatatgttctggtatcgacaagacctgggacatgggctgaggctgatccattactcatatggtgttcaagacactaacaaaggagaagtctcagatggctacagtgtctctagatcaaacacagaggacctccccctcactctggagtctgctgcctcctcccagacatctgtatatttctgcgccagcagtgagtc

SEQ ID NO: 208 - DNA, 344 bp, Artificial Sequence
  Synthetic Polynucleotide
atgggcaccaggctcttcttctatgtggccctttgtctgctgtgggcaggacacagggatgctggaatcacccagagcccaagatacaagatcacagagacaggaaggcaggtgaccttgatgtgtcaccagacttggagccacagctatatgttctggtatcgacaagacctgggacatgggctgaggctgatctattactcagcagctgctgatattacagataaaggagaagtccccgatggctatgttgtctccagatccaagacagagaatttccccctcactctggagtcagctacccgctcccagacatctgtgtatttctgcgccagcagtgagtc

SEQ ID NO: 209 - DNA, 344 bp, Artificial Sequence
  Synthetic Polynucleotide
atgggcacaaggttgttcttctatgtggccctttgtctcctgtggacaggacacatggatgctggaatcacccagagcccaagacacaaggtcacagagacaggaacaccagtgactctgagatgtcaccagactgagaaccaccgctatatgtactggtatcgacaagacccggggcatgggctgaggctgatccattactcatatggtgttaaagatactgacaaaggagaagtctcagatggctatagtgtctctagatcaaagacagaggatttcctcctcactctggagtccgctaccagctcccagacatctgtgtacttctgtgccatcagtgagtc

SEQ ID NO: 210 - DNA, 347 bp, Artificial Sequence
  Synthetic Polynucleotide
atgagcaccaggcttctctgctggatggccctctgtctcctgggggcagaactctcagaagctgaagttgcccagtcccccagatataagattacagagaaaagccaggctgtggctttttggtgtgatcctatttctggccatgctaccctttactggtaccggcagatcctgggacagggcccggagcttctggttcaatttcaggatgagagtgtagtagatgattcacagttgcctaaggatcgattttctgcagagaggctcaaaggagtagactccactctcaagatccagcctgcagagcttggggactcggccatgtatctctgtgccagcagcttagc

SEQ ID NO: 211 - DNA, 347 bp, Artificial Sequence
  Synthetic Polynucleotide
atgggcaccaggctcctctgctgggcggccctctgtctcctgggagcagaactcacagaagctggagttgcccagtctcccagatataagattatagagaaaaggcagagtgtggctttttggtgcaatcctatatctggccatgctaccctttactggtaccagcagatcctgggacagggcccaaagcttctgattcagtttcagaataacggtgtagtggatgattcacagttgcctaaggatcgattttctgcagagaggctcaaaggagtagactccactctcaagatccagcctgcaaagcttgaggactcggccgtgtatctctgtgccagcagcttaga

SEQ ID NO: 212 - DNA, 347 bp, Artificial Sequence
  Synthetic Polynucleotide
atgggtaccaggctcctctgctgggtggccttctgtctcctggtggaagaactcatagaagctggagtggttcagtctcccagatataagattatagagaaaaaacagcctgtggctttttggtgcaatcctatttctggccacaataccctttactggtacctgcagaacttgggacagggcccggagcttctgattcgatatgagaatgaggaagcagtagacgattcacagttgcctaaggatcgattttctgcagagaggctcaaaggagtagactccactctcaagatccagcctgcagagcttggggactcggccgtgtatctctgtgccagcagcttaga

SEQ ID NO: 213 - DNA, 344 bp, Artificial Sequence
  Synthetic Polynucleotide
atgggctcttggaccctctgtgtgtccctttatatcctggtagcgacacacacagatgctggtgttatccagtcacccaggcacaaagtgacagagatgggacaatcagtaactctgagatgcgaaccaatttcaggccacaatgatcttctctggtacagacagacctttgtgcagggactggaattgctgaattacttctgcagctggaccctcgtagatgactcaggagtgtccaaggattgattctcagcacagatgcctgatgtatcattctccactctgaggatccagcccatggaacccagggacttgggcctatatttctgtgccagcagctttgc

SEQ ID NO: 214 - DNA, 344 bp, Artificial Sequence
  Synthetic Polynucleotide
atggactcctggaccctctgtgtgtccctttgtatcctggtagcgacatgcacagatgctggcattatccagtcacccaagcatgaggtgacagaaatgggacaaacagtgactctgagatgtgagccaatttttggccacaatttccttttctggtacagagataccttcgtgcagggactggaattgctgagttacttccggagctgatctattatagataatgcaggtatgcccacagagcgattctcagctgagaggcctgatggatcattctctactctgaagatccagcctgcagagcagggggactcggccgtgtatgtctgtgcaagtcgcttagc

SEQ ID NO: 215 - DNA, 347 bp, Artificial Sequence
  Synthetic Polynucleotide
atggactcctggaccttctgctgtgtgtccctttgcatcctggtagcgaagcatacagatgctggagttatccagtcaccccgccatgaggtgacagagatgggacaagaagtgactctgagatgtaaaccaatttcaggccacaactcccttttctggtacagacagaccatgatgcggggactggagttgctcatttactttaacaacaacgttccgatagatgattcagggatgcccgaggatcgattctcagctaagatgcctaatgcatcattctccactctgaagatccagccctcagaacccagggactcagctgtgtacttctgtgccagcagtttagc

SEQ ID NO: 216 - DNA, 347 bp, Artificial Sequence
  Synthetic Polynucleotide
atgggctcctggaccctctgctgtgtgtccctttgcatcctggtagcaaagcacacagatgctggagttatccagtcaccccggcacgaggtgacagagatgggacaagaagtgactctgagatgtaaaccaatttcaggacacgactaccttttctggtacagacagaccatgatgcggggactggagttgctcatttactttaacaacaacgttccgatagatgattcagggatgcccgaggatcgattctcagctaagatgcctaatgcatcattctccactctgaagatccagccctcagaacccagggactcagctgtgtacttctgtgccagcagtttagc

SEQ ID NO: 217 - DNA, 347 bp, Artificial Sequence
  Synthetic Polynucleotide
atggccaccaggctcctctgctgtgtggttctttgtctcctgggagaagagcttatagatgctagagtcacccagacaccaaggcacaaggtgacagagatgggacaagaagtaacaatgagatgtcagccaattttaggccacaatactgttttctggtacagacagaccatgatgcaaggactggagttgctggcttacttccgcaaccgggctcctctagatgattcggggatgccgaaggatcgattctcagcagagatgcctgatgcaactttagccactctgaagatccagccctcagaacccagggactcagctgtgtatttttgtgctagtggtttggt

SEQ ID NO: 218 - DNA, 374 bp, Artificial Sequence
  Synthetic Polynucleotide
atgcttagtcctgacctgcctgactctgcctggaacaccaggctcctctgccatgtcatgctttgtctcctgggagcagtttcagtggctgctggagtcatccagtccccaagacatctgatcaaagaaaagagggaaacagccactctgaaatgctatcctatccctagacacgacactgtctactggtaccagcagggtccaggtcaggacccccagttcctcatttcgttttatgaaaagatgcagagcgataaaggaagcatccctgatcgattctcagctcaacagttcagtgactatcattctgaactgaacatgagctccttggagctgggggactcagccctgtacttctgtgccagcagcttagg

SEQ ID NO: 219 - DNA, 347 bp, Artificial Sequence
  Synthetic Polynucleotide
atggtttccaggcttctcagtttagtgtccctttgtctcctgggagcaaagcacatagaagctggagttactcagttccccagccacagcgtaatagagaagggccagactgtgactctgagatgtgacccaatttctggacatgataatctttattggtatcgacgtgttatgggaaaagaaataaaatttctgttacattttgtgaaagagtctaaacaggatgagtccggtatgcccaacaatcgattcttagctgaaaggactggagggacgtattctactctgaaggtgcagcctgcagaactggaggattctggagtttatttctgtgccagcagccaaga

SEQ ID NO: 220 - DNA, 344 bp, Artificial Sequence
  Synthetic Polynucleotide
atgggtcctgggcttctccactggatggccctttgtctccttggaacaggtcatggggatgccatggtcatccagaacccaagataccaggttacccagtttggaaagccagtgaccctgagttgttctcagactttgaaccataacgtcatgtactggtaccagcagaagtcaagtcaggccccaaagctgctgttccactactatgacaaagattttaacaatgaagcagacacccctgataacttccaatccaggaggccgaacacttctttctgctttcttgacatccgctcaccaggcctgggggacacagccatgtacctgtgtgccaccagcagaga

SEQ ID NO: 221 - DNA, 347 bp, Artificial Sequence
  Synthetic Polynucleotide
atgagcccaatattcacctgcatcacaatcctttgtctgctggctgcaggttctcctggtgaagaagtcgcccagactccaaaacatcttgtcagaggggaaggacagaaagcaaaattatattgtgccccaataaaaggacacagttatgttttttggtaccaacaggtcctgaaaaacgagttcaagttcttgatttccttccagaatgaaaatgtctttgatgaaacaggtatgcccaaggaaagattttcagctaagtgcctcccaaattcaccctgtagccttgagatccaggctacgaagcttgaggattcagcagtgtatttttgtgccagcagccaatc

SEQ ID NO: 222 - DNA, 344 bp, Artificial Sequence
  Synthetic Polynucleotide
atggatatctggctcctctgctgggtgaccctgtgtctcttggcggcaggacactcggagcctggagtcagccagacccccagacacaaggtcaccaacatgggacaggaggtgattctgaggtgcgatccatcttctggtcacatgtttgttcactggtaccgacagaatctgaggcaagaaatgaagttgctgatttccttccagtaccaaaacattgcagttgattcagggatgcccaaggaacgattcacagctgaaagacctaacggaacgtcttccacgctgaagatccatcccgcagagccgagggactcagccgtgtatctctacagtagcggtgg

SEQ ID NO: 223 - DNA, 347 bp, Artificial Sequence
  Synthetic Polynucleotide
atggacaccagagtactctgctgtgcggtcatctgtcttctgggggcaggtctctcaaatgccggcgtcatgcagaacccaagacacctggtcaggaggaggggacaggaggcaagactgagatgcagcccaatgaaaggacacagtcatgtttactggtatcggcagctcccagaggaaggtctgaaattcatggtttatctccagaaagaaaatatcatagatgagtcaggaatgccaaaggaacgattttctgctgaatttcccaaagagggccccagcatcctgaggatccagcaggtagtgcgaggagattcggcagcttatttctgtgccagctcaccacc

SEQ ID NO: 224 - DNA, 344 bp, Artificial Sequence
  Synthetic Polynucleotide
atgagcaaccaggtgctctgctgtgtggtcctttgtttcctgggagcaaacaccgtggatggtggaatcactcagtccccaaagtacctgttcagaaaggaaggacagaatgtgaccctgagttgtgaacagaatttgaaccacgatgccatgtactggtaccgacaggacccagggcaagggctgagattgatctactactcacagatagtaaatgactttcagaaaggagatatagctgaagggtacagcgtctctcgggagaagaaggaatcctttcctctcactgtgacatcggcccaaaagaacccgacagctttctatctctgtgccagtagtataga

SEQ ID NO: 225 - DNA, 368 bp, Artificial Sequence
  Synthetic Polynucleotide
atgctgctgcttctgctgcttctggggccaggtataagcctccttctacctgggagcttggcaggctccgggcttggtgctgtcgtctctcaacatccgagctgggttatctgtaagagtggaacctctgtgaagatcgagtgccgttccctggactttcaggccacaactatgttttggtatcgtcagttcccgaaacagagtctcatgctgatggcaacttccaatgagggctccaaggccacatacgagcaaggcgtcgagaaggacaagtttctcatcaaccatgcaagcctgaccttgtccactctgacagtgaccagtgcccatcctgaagacagcagcttctacatctgcagtgctagaga

SEQ ID NO: 226 - DNA, 348 bp, Artificial Sequence
  Synthetic Polynucleotide
atgtgcctcagacttctctgctgtgtggccatttctttctggggagccaggctccacggacaccaaggtcacccagagacctagacttctggtcaaagcaagtgaacagaaagcaaagatggattgtgttcctataaaagcacatagttatgtttactggtatcgtaagaagctggaagaagagctcaagtttttggtttactttcagaatgaagaacttattcagaaagcagaaataatcaatgagcgatttttagcccaatgctccaaaaactcatcctgtaccttggagatccagtccacggagtcaggggacacagcactgtatttctgtgccagcagcaaagc

SEQ ID NO: 227 - DNA, 345 bp, Artificial Sequence
  Synthetic Polynucleotide
atggggagctgggtcctctgctatgtgaccctgtgtctcctgggagcaggacccttggatgctgacatctatcagatgccattccagctcactggggctggatgggatgtgactctggagtggaaacggaatttgagacacaatgacatgtactgctactggtactggcaggacccaaagcaaaatctgagactgatctattactcaagggttgaaaaggatattcagagaggagatctaactgaaggctacgtgtctgccaagaggagaaggggctatttcttctcagggtgaagttggcccacaccagccaaacagctttgtacttctgtcctgggagcgcac

SEQ ID NO: 228 - DNA, 347 bp, Artificial Sequence
  Synthetic Polynucleotide
atgggcaccaggctcctcggctgtgcagccctgtgtctcctggcagcagactcttttcatgccaaagtcacacagactccaggacatttggtcaaaggaaaaggacagaaaacaaagatggattgtacccccgaaaaaggacatacttttgtttattggtatcaacagaatcagaataaagagtttatgcttttgatttcctttcagaatgaacaagttcttcaagaaacggagatgcacaagaagcgattctcatctcaatgccccaagaacgcaccctgcagcctggcaatcctgtcctcagaaccgggagacacggcactgtatctctgcgccagcagtcaatc

SEQ ID NO: 229 - DNA, 345 bp, Artificial Sequence
  Synthetic Polynucleotide
atggcctccctgctcttcttctgtggggccttttatctcctgggaacagggtccatggatgctgatgttacccagaccccaaggaataggatcacaaagacaggaaagaggattatgctggaatgttctcagactaagggtcatgatagaatgtactggtatcgacaagacccaggactgggcctacggttgatctattactcctttgatgtcaaagatataaacaaaggagagatctctgatggatacagtgtctctcgacaggcacaggctaaattctccctgtccctagagtctgccatccccaaccagacagctctttacttctgtgccaccagtgatttg

SEQ ID NO: 230 - DNA, 344 bp, Artificial Sequence
  Synthetic Polynucleotide
atgactatcaggctcctctgctacatgggcttttattttctgggggcaggcctcatggaagctgacatctaccagaccccaagataccttgttatagggacaggaaagaagatcactctggaatgttctcaaaccatgggccatgacaaaatgtactggtatcaacaagatccaggaatggaactacacctcatccactattcctatggagttaattccacagagaagggagatctttcctctgagtcaacagtctccagaataaggacggagcattttcccctgaccctggagtctgccaggccctcacatacctctcagtacctctgtgccagcagtgaata

SEQ ID NO: 231 - DNA, 344 bp, Artificial Sequence
  Synthetic Polynucleotide
atgagcaacaggcttctctgctgtgtgatcatttgtctcctaagagcaggcctcaaggatgctgtagttacacaattcccaagacacagaatcattgggacaggaaaggaattcattctacagtgttcccagaatatgaatcatgttacaatgtactggtatcgacaggacccaggacttggactgaagctggtctattattcacctggcactgggagcactgaaaaaggagatatctctgaggggtatcatgtttcttgaaatactatagcatcttttcccctgaccctgaagtctgccagcaccaaccagacatctgtgtatctctatgccagcagttcatc

SEQ ID NO: 232 - DNA, 344 bp, Artificial Sequence
  Synthetic Polynucleotide
atgggcccccagctccttggctatgtggtcctttgccttctaggagcaggccccctggaagcccaagtgacccagaacccaagatacctcatcacagtgactggaaagaagttaacagtgacttgttctcagaatatgaaccatgagtatatgtcctggtatcgacaagacccagggctgggcttaaggcagatctactattcaatgaatgttgaggtgactgataagggagatgttcctgaagggtacaaagtctctcgaaaagagaagaggaatttccccctgatcctggagtcgcccagccccaaccagacctctctgtacttctgtgccagcagtttatc

SEQ ID NO: 233 - DNA, 344 bp, Artificial Sequence
  Synthetic Polynucleotide
atgggaatcaggctcctgtgtcgtgtggccttttgtttcctggctgtaggcctcgtagatgtgaaagtaacccagagctcgagatatctagtcaaaaggacgggagagaaagtttttctggaatgtgtccaggatatggaccatgaaaatatgttctggtatcgacaagacccaggtctggggctacggctgatctatttctcatatgatgttaaaatgaaagaaaaaggagatattcctgaggggtacagtgtctctagagagaagaaggagcgcttctccctgattctggagtccgccagcaccaaccagacatctatgtacctctgtgccagcagtttatg

SEQ ID NO: 234 - DNA, 335 bp, Artificial Sequence
  Synthetic Polynucleotide
atgctgagtcttctgctccttctcctgggactaggctctgtgttcagtgctgtcatctctcaaaagccaagcagggatatctgtcaacgtggaacctccctgacgatccagtgtcaagtcgatagccaagtcaccatgatgttctggtaccgtcagcaacctggacagagcctgacactgatcgcaactgcaaatcagggctctgaggccacatatgagagtggatttgtcattgacaagtttcccatcagccgcccaaacctaacattctcaactctgactgtgagcaacatgagccctgaagacagcagcatatatctctgcagcgttgaaga

SEQ ID NO: 235 - DNA, 335 bp, Artificial Sequence
  Synthetic Polynucleotide
atgctctgctctctccttgcccttctcctgggcactttctttggggtcagatctcagactattcatcaatggccagcgaccctggtgcagcctgtgggcagcccgctctctctggagtgcactgtggagggaacatcaaaccccaacctatactggtaccgacaggctgcaggcaggggcctccagctgctcttctactccgttggtattggccagatcagctctgaggtgccccagaatctctcagcctccagaccccaggaccggcagttcatcctgagttctaagaagctccttctcagtgactctggcttctatctctgtgcctggagtgt

SEQ ID NO: 236 - protein, 9 aa, Artificial Sequence
  Synthetic Polypeptide
TEDYMIHII

SEQ ID NO: 237 - protein, 16 aa, Artificial Sequence
  Synthetic Polypeptide
CASSRHVGGVPEAFFG

SEQ ID NO: 238 - protein, 14 aa, Artificial Sequence
  Synthetic Polypeptide
CASSIGRGSEQYFG

SEQ ID NO: 239 - protein, 14 aa, Artificial Sequence
  Synthetic Polypeptide
CASSDVLSGEAFFG

SEQ ID NO: 240 - protein, 14 aa, Artificial Sequence
  Synthetic Polypeptide
CASQGHKNTEAFFG

SEQ ID NO: 241 - protein, 19 aa, Artificial Sequence
  Synthetic Polypeptide
CASSLGPGGVKTNEKLFFG

SEQ ID NO: 242 - protein, 19 aa, Artificial Sequence
  Synthetic Polypeptide
CASSLGPGGVKTNEKLFFG

SEQ ID NO: 243 - protein, 14 aa, Artificial Sequence
  Synthetic Polypeptide
CASSDVLSGEAFFG

SEQ ID NO: 244 - protein, 14 aa, Artificial Sequence
  Synthetic Polypeptide
CASQGHKNTEAFFG

SEQ ID NO: 245 - protein, 19 aa, Artificial Sequence
  Synthetic Polypeptide
CASSLGPGGVKTNEKLFFG

SEQ ID NO: 246 - protein, 14 aa, Artificial Sequence
  Synthetic Polypeptide
CASSIGRGSEQYFG

SEQ ID NO: 247 - protein, 16 aa, Artificial Sequence
  Synthetic Polypeptide
CASSRHVGGVPEAFFG

SEQ ID NO: 248 - protein, 14 aa, Artificial Sequence
  Synthetic Polypeptide
CASSASKGQPQHFG

SEQ ID NO: 249 - protein, 14 aa, Artificial Sequence
  Synthetic Polypeptide
CASQGHKNTEAFFG

SEQ ID NO: 250 - protein, 19 aa, Artificial Sequence
  Synthetic Polypeptide
CASSLGPGGVKTNEKLFFG

SEQ ID NO: 251 - DNA, 43 bp, Artificial Sequence
  Synthetic Polynucleotide
aaacgacggccagtgaattgtaatacgactcactataggcgct

SEQ ID NO: 252 - DNA, 40 bp, Artificial Sequence
  Synthetic Polynucleotide
ggccagtgaattgtaatacgactcactatagggaggcggt

SEQ ID NO: 253 - DNA, 27 bp, Artificial Sequence
  Synthetic Polynucleotide
taatacgactcactatagggaggcggt

SEQ ID NO: 254 - DNA, 30 bp, Artificial Sequence
  Synthetic Polynucleotide
ggtaatacgactcactatagggagaagagt

SEQ ID NO: 255 - DNA, 27 bp, Artificial Sequence
  Synthetic Polynucleotide
aattaatacgactcactatagggagat

SEQ ID NO: 256 - DNA, 14 bp, Artificial Sequence
  Synthetic polynucleotide
tcgtcggcagcgtc

SEQ ID NO: 257 - DNA, 58 bp, Artificial Sequence
  Synthetic polynucleotide
gtctcgtgggctcggagatgtgtataagagacaggaatcaaaatcggtgaataggcag

SEQ ID NO: 258 - DNA, 59 bp, Artificial Sequence
  Synthetic polynucleotide
gtctcgtgggctcggagatgtgtataagagacaggccaggcacaccagtgtggcctttt

SEQ ID NO: 259 - DNA, 37 bp, Artificial Sequence
  Synthetic polynucleotide
caagcagaagacggcatacgagatgtctcgtgggctc

SEQ ID NO: 260 - DNA, 41 bp, Artificial Sequence
  Synthetic polynucleotide
aatgatacggcgaccaccgagatctacactcgtcggcagcg

SEQ ID NO: 261 - DNA, 67 bp, Artificial Sequence
  Synthetic polynucleotide
  misc_feature (39)..(42): n is a, c, g, or t
tcgtcggcagcgtcagatgtgtataagagacaghhhhhnnnncttctacaggagctccagatgaaag

SEQ ID NO: 262 - DNA, 67 bp, Artificial Sequence
  Synthetic polynucleotide
  misc_feature (39)..(42): n is a, c, g, or t
tcgtcggcagcgtcagatgtgtataagagacaghhhhhnnnncttttgaaggagctccagatgaaag

SEQ ID NO: 263 - DNA, 64 bp, Artificial Sequence
  Synthetic polynucleotide
  misc_feature (39)..(42): n is a, c, g, or t
tcgtcggcagcgtcagatgtgtataagagacaghhhhhnnnntgctcatcctccaggtgcggga

SEQ ID NO: 264 - DNA, 65 bp, Artificial Sequence
  Synthetic polynucleotide
  misc_feature (39)..(42): n is a, c, g, or t
tcgtcggcagcgtcagatgtgtataagagacaghhhhhnnnngaagaaaccatctgcccttgtga

SEQ ID NO: 265 - DNA, 67 bp, Artificial Sequence
  Synthetic polynucleotide
  misc_feature (39)..(42): n is a, c, g, or t
tcgtcggcagcgtcagatgtgtataagagacaghhhhhnnnncctgccccgggtttccctgagcgac

SEQ ID NO: 266 - DNA, 65 bp, Artificial Sequence
  Synthetic polynucleotide
  misc_feature (39)..(42): n is a, c, g, or t
tcgtcggcagcgtcagatgtgtataagagacaghhhhhnnnntctctgcgcattgcagacaccca

SEQ ID NO: 267 - DNA, 65 bp, Artificial Sequence
  Synthetic polynucleotide
  misc_feature (39)..(42): n is a, c, g, or t
tcgtcggcagcgtcagatgtgtataagagacaghhhhhnnnnttgtttcatatcacagcctccca

SEQ ID NO: 268 - DNA, 64 bp, Artificial Sequence
  Synthetic polynucleotide
  misc_feature (39)..(42): n is a, c, g, or t
tcgtcggcagcgtcagatgtgtataagagacaghhhhhnnnngcttgtacattacagccgtgca

SEQ ID NO: 269 - DNA, 64 bp, Artificial Sequence
  Synthetic polynucleotide
  misc_feature (39)..(42): n is a, c, g, or t
tcgtcggcagcgtcagatgtgtataagagacaghhhhhnnnnatctgaggaaaccctctgtgca

SEQ ID NO: 270 - DNA, 65 bp, Artificial Sequence
  Synthetic polynucleotide
  misc_feature (39)..(42): n is a, c, g, or t
tcgtcggcagcgtcagatgtgtataagagacaghhhhhnnnnacctgacgaaaccctcagcccat

SEQ ID NO: 271 - DNA, 66 bp, Artificial Sequence
  Synthetic polynucleotide
  misc_feature (39)..(42): n is a, c, g, or t
tcgtcggcagcgtcagatgtgtataagagacaghhhhhnnnncctatgcctgtctttactttaatc

SEQ ID NO: 272 - DNA, 66 bp, Artificial Sequence
  Synthetic polynucleotide
  misc_feature (39)..(42): n is a, c, g, or t
tcgtcggcagcgtcagatgtgtataagagacaghhhhhnnnncttgaggaaaccctcagtccatat

SEQ ID NO: 273 - DNA, 66 bp, Artificial Sequence
  Synthetic polynucleotide
  misc_feature (39)..(42): n is a, c, g, or t
tcgtcggcagcgtcagatgtgtataagagacaghhhhhnnnngaaaccatcaacccatgtgagtga

SEQ ID NO: 274 - DNA, 65 bp, Artificial Sequence
  Synthetic polynucleotide
  misc_feature (39)..(42): n is a, c, g, or t
tcgtcggcagcgtcagatgtgtataagagacaghhhhhnnnnacttggagaaagactcagttcaa

SEQ ID NO: 275 - DNA, 65 bp, Artificial Sequence
  Synthetic polynucleotide
  misc_feature (39)..(42): n is a, c, g, or t
tcgtcggcagcgtcagatgtgtataagagacaghhhhhnnnnacttggagaaaggctcagttcaa

SEQ ID NO: 276 - DNA, 62 bp, Artificial Sequence
  Synthetic polynucleotide
  misc_feature (39)..(42): n is a, c, g, or t
tcgtcggcagcgtcagatgtgtataagagacaghhhhhnnnnctgcacatcacagcctccca

SEQ ID NO: 277 - DNA, 66 bp, Artificial Sequence
  Synthetic polynucleotide
  misc_feature (39)..(42): n is a, c, g, or t
tcgtcggcagcgtcagatgtgtataagagacaghhhhhnnnngtttggaatatcgcagcctctcat

SEQ ID NO: 278 - DNA, 65 bp, Artificial Sequence
  Synthetic polynucleotide
  misc_feature (39)..(42): n is a, c, g, or t
tcgtcggcagcgtcagatgtgtataagagacaghhhhhnnnnccctgctcatcagagactccaag

SEQ ID NO: 279 - DNA, 65 bp, Artificial Sequence
  Synthetic polynucleotide
  misc_feature (39)..(42): n is a, c, g, or t
tcgtcggcagcgtcagatgtgtataagagacaghhhhhnnnnctctgctcatcagagactcccag

SEQ ID NO: 280 - DNA, 65 bp, Artificial Sequence
  Synthetic polynucleotide
  misc_feature (39)..(42): n is a, c, g, or t
tcgtcggcagcgtcagatgtgtataagagacaghhhhhnnnnccttgttcatcagagactcacag

SEQ ID NO: 281 - DNA, 66 bp, Artificial Sequence
  Synthetic polynucleotide
  misc_feature (39)..(42): n is a, c, g, or t
tcgtcggcagcgtcagatgtgtataagagacaghhhhhnnnntccctgcacatcacagagacccaa

SEQ ID NO: 282 - DNA, 66 bp, Artificial Sequence
  Synthetic polynucleotide
  misc_feature (39)..(42): n is a, c, g, or t
tcgtcggcagcgtcagatgtgtataagagacaghhhhhnnnntctctgcaaattgcagctactcaa

SEQ ID NO: 283 - DNA, 66 bp, Artificial Sequence
  Synthetic polynucleotide
  misc_feature (39)..(42): n is a, c, g, or t
tcgtcggcagcgtcagatgtgtataagagacaghhhhhnnnnttgtcatctccgcttcacaactgg

SEQ ID NO: 284 - DNA, 66 bp, Artificial Sequence
  Synthetic polynucleotide
  misc_feature (39)..(42): n is a, c, g, or t
tcgtcggcagcgtcagatgtgtataagagacaghhhhhnnnngttttgaatatgctggtctctcat

SEQ ID NO: 285 - DNA, 66 bp, Artificial Sequence
  Synthetic polynucleotide
  misc_feature (39)..(42): n is a, c, g, or t
tcgtcggcagcgtcagatgtgtataagagacaghhhhhnnnncctgaagaaaccatttgctcaaga

SEQ ID NO: 286 - DNA, 66 bp, Artificial Sequence
  Synthetic polynucleotide
  misc_feature (39)..(42): n is a, c, g, or t
tcgtcggcagcgtcagatgtgtataagagacaghhhhhnnnntccttgttgatcacggcttcccgg

SEQ ID NO: 287 - DNA, 64 bp, Artificial Sequence
  Synthetic polynucleotide
  misc_feature (39)..(42): n is a, c, g, or t
tcgtcggcagcgtcagatgtgtataagagacaghhhhhnnnnacctggagaagccctcggtgca

SEQ ID NO: 288 - DNA, 66 bp, Artificial Sequence
  Synthetic polynucleotide
  misc_feature (39)..(42): n is a, c, g, or t
tcgtcggcagcgtcagatgtgtataagagacaghhhhhnnnncaccatcacagcctcacaagtcgt

SEQ ID NO: 289 - DNA, 64 bp, Artificial Sequence
  Synthetic polynucleotide
  misc_feature (39)..(42): n is a, c, g, or t
tcgtcggcagcgtcagatgtgtataagagacaghhhhhnnnntttctgcacatcacagccccta

SEQ ID NO: 290 - DNA, 67 bp, Artificial Sequence
  Synthetic polynucleotide
  misc_feature (39)..(42): n is a, c, g, or t
tcgtcggcagcgtcagatgtgtataagagacaghhhhhnnnnctttatacattgcagcttctcagcc

SEQ ID NO: 291 - DNA, 66 bp, Artificial Sequence
  Synthetic polynucleotide
  misc_feature (39)..(42): n is a, c, g, or t
tcgtcggcagcgtcagatgtgtataagagacaghhhhhnnnngtacatttcctcttcccagaccac

SEQ ID NO: 292 - DNA, 66 bp, Artificial Sequence
  Synthetic polynucleotide
  misc_feature (39)..(42): n is a, c, g, or t
tcgtcggcagcgtcagatgtgtataagagacaghhhhhnnnncattgcatatcatggattcccagc

SEQ ID NO: 293 - DNA, 66 bp, Artificial Sequence
  Synthetic polynucleotide
  misc_feature (39)..(42): n is a, c, g, or t
tcgtcggcagcgtcagatgtgtataagagacaghhhhhnnnngctatttgtacatcaaaggatccc

SEQ ID NO: 294 - DNA, 65 bp, Artificial Sequence
  Synthetic polynucleotide
  misc_feature (39)..(42): n is a, c, g, or t
tcgtcggcagcgtcagatgtgtataagagacaghhhhhnnnncagctccctgcacatcacagcca

SEQ ID NO: 295 - DNA, 67 bp, Artificial Sequence
  Synthetic polynucleotide
  misc_feature (39)..(42): n is a, c, g, or t
tcgtcggcagcgtcagatgtgtataagagacaghhhhhnnnnttgatcctgccccacgctacgctga

SEQ ID NO: 296 - DNA, 67 bp, Artificial Sequence
  Synthetic polynucleotide
  misc_feature (39)..(42): n is a, c, g, or t
tcgtcggcagcgtcagatgtgtataagagacaghhhhhnnnnttgatcctgcaccgtgctaccttga

SEQ ID NO: 297 - DNA, 65 bp, Artificial Sequence
  Synthetic polynucleotide
  misc_feature (39)..(42): n is a, c, g, or t
tcgtcggcagcgtcagatgtgtataagagacaghhhhhnnnngttctctccacatcactgcagcc

SEQ ID NO: 298 - DNA, 65 bp, Artificial Sequence
  Synthetic polynucleotide
  misc_feature (39)..(42): n is a, c, g, or t
tcgtcggcagcgtcagatgtgtataagagacaghhhhhnnnngccacctatacatcagattccca

SEQ ID NO: 299 - DNA, 65 bp, Artificial Sequence
  Synthetic polynucleotide
  misc_feature (39)..(42): n is a, c, g, or t
tcgtcggcagcgtcagatgtgtataagagacaghhhhhnnnntctctgcacattgtgccctccca

SEQ ID NO: 300 - DNA, 67 bp, Artificial Sequence
  Synthetic polynucleotide
  misc_feature (39)..(42): n is a, c, g, or t
tcgtcggcagcgtcagatgtgtataagagacaghhhhhnnnnccctgtaccttacggcctcccagct

SEQ ID NO: 301 - DNA, 66 bp, Artificial Sequence
  Synthetic polynucleotide
  misc_feature (39)..(42): n is a, c, g, or t
tcgtcggcagcgtcagatgtgtataagagacaghhhhhnnnncttatcatatcatcatcacagcca

SEQ ID NO: 302 - DNA, 66 bp, Artificial Sequence
  Synthetic polynucleotide
  misc_feature (39)..(42): n is a, c, g, or t
tcgtcggcagcgtcagatgtgtataagagacaghhhhhnnnntccctgcatattacagccacccaa

SEQ ID NO: 303 - DNA, 66 bp, Artificial Sequence
  Synthetic polynucleotide
  misc_feature (39)..(42): n is a, c, g, or t
tcgtcggcagcgtcagatgtgtataagagacaghhhhhnnnnacctcaccatcaattccttaaaac

SEQ ID NO: 304 - DNA, 66 bp, Artificial Sequence
  Synthetic polynucleotide
  misc_feature (39)..(42): n is a, c, g, or t
tcgtcggcagcgtcagatgtgtataagagacaghhhhhnnnntccctgcatatcacagcctcccag

SEQ ID NO: 305 - DNA, 66 bp, Artificial Sequence
  Synthetic polynucleotide
  misc_feature (39)..(42): n is a, c, g, or t
tcgtcggcagcgtcagatgtgtataagagacaghhhhhnnnncttcctgaatatctcagcatccat

SEQ ID NO: 306 - DNA, 65 bp, Artificial Sequence
  Synthetic polynucleotide
  misc_feature (39)..(42): n is a, c, g, or t
tcgtcggcagcgtcagatgtgtataagagacaghhhhhnnnntcctgaacatcacagccacccag

SEQ ID NO: 307 - DNA, 66 bp, Artificial Sequence
  Synthetic polynucleotide
  misc_feature (39)..(42): n is a, c, g, or t
tcgtcggcagcgtcagatgtgtataagagacaghhhhhnnnntccctgcacatacaggattcccag

SEQ ID NO: 308 - DNA, 65 bp, Artificial Sequence
  Synthetic polynucleotide
  misc_feature (39)..(42): n is a, c, g, or t
tcgtcggcagcgtcagatgtgtataagagacaghhhhhnnnncaagatctcagactcacagctgg

SEQ ID NO: 309 - DNA, 65 bp, Artificial Sequence
  Synthetic polynucleotide
  misc_feature (39)..(42): n is a, c, g, or t
tcgtcggcagcgtcagatgtgtataagagacaghhhhhnnnnccgtctcagcaccctccacatca

SEQ ID NO: 310 - DNA, 66 bp, Artificial Sequence
  Synthetic polynucleotide
  misc_feature (39)..(42): n is a, c, g, or t
tcgtcggcagcgtcagatgtgtataagagacaghhhhhnnnnccattgtgaaatattcagtccagg

SEQ ID NO: 311 - DNA, 65 bp, Artificial Sequence
  Synthetic polynucleotide
  misc_feature (39)..(42): n is a, c, g, or t
tcgtcggcagcgtcagatgtgtataagagacaghhhhhnnnngtggtcgcactgcagcaagaaga

SEQ ID NO: 312 - DNA, 66 bp, Artificial Sequence
  Synthetic polynucleotide
  misc_feature (39)..(42): n is a, c, g, or t
tcgtcggcagcgtcagatgtgtataagagacaghhhhhnnnngatccggtccacaaagctggagga

SEQ ID NO: 313 - DNA, 66 bp, Artificial Sequence
  Synthetic polynucleotide
  misc_feature (39)..(42): n is a, c, g, or t
tcgtcggcagcgtcagatgtgtataagagacaghhhhhnnnncatcaattccctggagcttggtga

SEQ ID NO: 314 - DNA, 66 bp, Artificial Sequence
  Synthetic polynucleotide
  misc_feature (39)..(42): n is a, c, g, or t
tcgtcggcagcgtcagatgtgtataagagacaghhhhhnnnnttcacctacacgccctgcagccag

SEQ ID NO: 315 - DNA, 66 bp, Artificial Sequence
  Synthetic polynucleotide
  misc_feature (39)..(42): n is a, c, g, or t
tcgtcggcagcgtcagatgtgtataagagacaghhhhhnnnnttcacctacacaccctgcagccag

SEQ ID NO: 316 - DNA, 65 bp, Artificial Sequence
  Synthetic polynucleotide
  misc_feature (39)..(42): n is a, c, g, or t
tcgtcggcagcgtcagatgtgtataagagacaghhhhhnnnngaatgtgagcaccttggagctgg

SEQ ID NO: 317 - DNA, 66 bp, Artificial Sequence
  Synthetic polynucleotide
  misc_feature (39)..(42): n is a, c, g, or t
tcgtcggcagcgtcagatgtgtataagagacaghhhhhnnnntactgagtcaaacacggagctagg

SEQ ID NO: 318 - DNA, 66 bp, Artificial Sequence
  Synthetic polynucleotide
  misc_feature (39)..(42): n is a, c, g, or t
tcgtcggcagcgtcagatgtgtataagagacaghhhhhnnnngctctgagatgaatgtgagtgcct

SEQ ID NO: 319 - DNA, 64 bp, Artificial Sequence
  Synthetic polynucleotide
  misc_feature (39)..(42): n is a, c, g, or t
tcgtcggcagcgtcagatgtgtataagagacaghhhhhnnnnctgagctgaatgtgaacgcctt

SEQ ID NO: 320 - DNA, 64 bp, Artificial Sequence
  Synthetic polynucleotide
  misc_feature (39)..(42): n is a, c, g, or t
tcgtcggcagcgtcagatgtgtataagagacaghhhhhnnnngagttctcgctcaggctggagt

SEQ ID NO: 321 - DNA, 64 bp, Artificial Sequence
  Synthetic polynucleotide
  misc_feature (39)..(42): n is a, c, g, or t
tcgtcggcagcgtcagatgtgtataagagacaghhhhhnnnnctggggttggagtcggctgctc

SEQ ID NO: 322 - DNA, 64 bp, Artificial Sequence
  Synthetic polynucleotide
  misc_feature (39)..(42): n is a, c, g, or t
tcgtcggcagcgtcagatgtgtataagagacaghhhhhnnnncccctcacgttggcgtctgctg

SEQ ID NO: 323 - DNA, 64 bp, Artificial Sequence
  Synthetic polynucleotide
  misc_feature (39)..(42): n is a, c, g, or t
tcgtcggcagcgtcagatgtgtataagagacaghhhhhnnnntcccgctcaggctgctgtcggc

SEQ ID NO: 324 - DNA, 64 bp, Artificial Sequence
  Synthetic polynucleotide
  misc_feature (39)..(42): n is a, c, g, or t
tcgtcggcagcgtcagatgtgtataagagacaghhhhhnnnngatttcccgctcaggctggagt

SEQ ID NO: 325 - DNA, 65 bp, Artificial Sequence
  Synthetic polynucleotide
  misc_feature (39)..(42): n is a, c, g, or t
tcgtcggcagcgtcagatgtgtataagagacaghhhhhnnnntccccctcaagctggagtcagct

SEQ ID NO: 326 - DNA, 64 bp, Artificial Sequence
  Synthetic polynucleotide
  misc_feature (39)..(42): n is a, c, g, or t
tcgtcggcagcgtcagatgtgtataagagacaghhhhhnnnntcccactcaggctggtgtcggc

SEQ ID NO: 327 - DNA, 64 bp, Artificial Sequence
  Synthetic polynucleotide
  misc_feature (39)..(42): n is a, c, g, or t
tcgtcggcagcgtcagatgtgtataagagacaghhhhhnnnnctctgaagttccagcgcacaca

SEQ ID NO: 328 - DNA, 64 bp, Artificial Sequence
  Synthetic polynucleotide
  misc_feature (39)..(42): n is a, c, g, or t
tcgtcggcagcgtcagatgtgtataagagacaghhhhhnnnngatccagcgcacacagcaggag

SEQ ID NO: 329 - DNA, 65 bp, Artificial Sequence
  Synthetic polynucleotide
  misc_feature (39)..(42): n is a, c, g, or t
tcgtcggcagcgtcagatgtgtataagagacaghhhhhnnnnactctgaagatccagcgcacaga

SEQ ID NO: 330 - DNA, 64 bp, Artificial Sequence
  Synthetic polynucleotide
  misc_feature (39)..(42): n is a, c, g, or t
tcgtcggcagcgtcagatgtgtataagagacaghhhhhnnnnagatccagcgcacagagcaagg

SEQ ID NO: 331 - DNA, 64 bp, Artificial Sequence
  Synthetic polynucleotide
  misc_feature (39)..(42): n is a, c, g, or t
tcgtcggcagcgtcagatgtgtataagagacaghhhhhnnnncagcgcacagagcagcgggact

SEQ ID NO: 332 - DNA, 64 bp, Artificial Sequence
  Synthetic polynucleotide
  misc_feature (39)..(42): n is a, c, g, or t
tcgtcggcagcgtcagatgtgtataagagacaghhhhhnnnngagatccagcgcacagagcagg

SEQ ID NO: 333 - DNA, 64 bp, Artificial Sequence
  Synthetic polynucleotide
  misc_feature (39)..(42): n is a, c, g, or t
tcgtcggcagcgtcagatgtgtataagagacaghhhhhnnnnccctcaaccctggagtctacta

SEQ ID NO: 334 - DNA, 64 bp, Artificial Sequence
  Synthetic polynucleotide
  misc_feature (39)..(42): n is a, c, g, or t
tcgtcggcagcgtcagatgtgtataagagacaghhhhhnnnntccccaatcctggcatccacca

SEQ ID NO: 335 - DNA, 65 bp, Artificial Sequence
  Synthetic polynucleotide
  misc_feature (39)..(42): n is a, c, g, or t
tcgtcggcagcgtcagatgtgtataagagacaghhhhhnnnnctaaacctgagctctctggagct

SEQ ID NO: 336 - DNA, 64 bp, Artificial Sequence
  Synthetic polynucleotide
  misc_feature (39)..(42): n is a, c, g, or t
tcgtcggcagcgtcagatgtgtataagagacaghhhhhnnnnccctcactctggagtctgctgc

SEQ ID NO: 337 - DNA, 64 bp, Artificial Sequence
  Synthetic polynucleotide
  misc_feature (39)..(42): n is a, c, g, or t
tcgtcggcagcgtcagatgtgtataagagacaghhhhhnnnnccctcactctggagtcagctac

SEQ ID NO: 338 - DNA, 64 bp, Artificial Sequence
  Synthetic polynucleotide
  misc_feature (39)..(42): n is a, c, g, or t
tcgtcggcagcgtcagatgtgtataagagacaghhhhhnnnntcctcactctggagtccgctac

SEQ ID NO: 339 - DNA, 65 bp, Artificial Sequence
  Synthetic polynucleotide
  misc_feature (39)..(42): n is a, c, g, or t
tcgtcggcagcgtcagatgtgtataagagacaghhhhhnnnnccactctcaagatccagcctgca

SEQ ID NO: 340 - DNA, 65 bp, Artificial Sequence
  Synthetic polynucleotide
  misc_feature (39)..(42): n is a, c, g, or t
tcgtcggcagcgtcagatgtgtataagagacaghhhhhnnnngaggatccagcccatggaaccca

SEQ ID NO: 341 - DNA, 64 bp, Artificial Sequence
  Synthetic polynucleotide
  misc_feature (39)..(42): n is a, c, g, or t
tcgtcggcagcgtcagatgtgtataagagacaghhhhhnnnnctgaagatccagcctgcagagc

SEQ ID NO: 342 - DNA, 64 bp, Artificial Sequence
  Synthetic polynucleotide
  misc_feature (39)..(42): n is a, c, g, or t
tcgtcggcagcgtcagatgtgtataagagacaghhhhhnnnncagccctcagaacccagggact

SEQ ID NO: 343 - DNA, 65 bp, Artificial Sequence
  Synthetic polynucleotide
  misc_feature (39)..(42): n is a, c, g, or t
tcgtcggcagcgtcagatgtgtataagagacaghhhhhnnnngagctccttggagctgggggact

SEQ ID NO: 344 - DNA, 64 bp, Artificial Sequence
  Synthetic polynucleotide
  misc_feature (39)..(42): n is a, c, g, or t
tcgtcggcagcgtcagatgtgtataagagacaghhhhhnnnnggtgcagcctgcagaactggag

SEQ ID NO: 345 - DNA, 64 bp, Artificial Sequence
  Synthetic polynucleotide
  misc_feature (39)..(42): n is a, c, g, or t
tcgtcggcagcgtcagatgtgtataagagacaghhhhhnnnngacatccgctcaccaggcctgg

SEQ ID NO: 346 - DNA, 64 bp, Artificial Sequence
  Synthetic polynucleotide
  misc_feature (39)..(42): n is a, c, g, or t
tcgtcggcagcgtcagatgtgtataagagacaghhhhhnnnntgagatccaggctacgaagctt

SEQ ID NO: 347 - DNA, 64 bp, Artificial Sequence
  Synthetic polynucleotide
  misc_feature (39)..(42): n is a, c, g, or t
tcgtcggcagcgtcagatgtgtataagagacaghhhhhnnnngaagatccatcccgcagagccg

SEQ ID NO: 348 - DNA, 64 bp, Artificial Sequence
  Synthetic polynucleotide
  misc_feature (39)..(42): n is a, c, g, or t
tcgtcggcagcgtcagatgtgtataagagacaghhhhhnnnnggatccagcaggtagtgcgagg

SEQ ID NO: 349 - DNA, 64 bp, Artificial Sequence
  Synthetic polynucleotide
  misc_feature (39)..(42): n is a, c, g, or t
tcgtcggcagcgtcagatgtgtataagagacaghhhhhnnnncactgtgacatcggcccaaaag

SEQ ID NO: 350 - DNA, 64 bp, Artificial Sequence
  Synthetic polynucleotide
  misc_feature (39)..(42): n is a, c, g, or t
tcgtcggcagcgtcagatgtgtataagagacaghhhhhnnnnctgacagtgaccagtgcccatc

SEQ ID NO: 351 - DNA, 64 bp, Artificial Sequence
  Synthetic polynucleotide
  misc_feature (39)..(42): n is a, c, g, or t
tcgtcggcagcgtcagatgtgtataagagacaghhhhhnnnngagatccagtccacggagtcag

SEQ ID NO: 352 - DNA, 65 bp, Artificial Sequence
  Synthetic polynucleotide
  misc_feature (39)..(42): n is a, c, g, or t
tcgtcggcagcgtcagatgtgtataagagacaghhhhhnnnngtgaagttggcccacaccagcca

SEQ ID NO: 353 - DNA, 64 bp, Artificial Sequence
  Synthetic polynucleotide
  misc_feature (39)..(42): n is a, c, g, or t
tcgtcggcagcgtcagatgtgtataagagacaghhhhhnnnncctggcaatcctgtcctcagaa

SEQ ID NO: 354 - DNA, 64 bp, Artificial Sequence
  Synthetic polynucleotide
  misc_feature (39)..(42): n is a, c, g, or t
tcgtcggcagcgtcagatgtgtataagagacaghhhhhnnnngagtctgccatccccaaccaga

SEQ ID NO: 355 - DNA, 63 bp, Artificial Sequence
  Synthetic polynucleotide
  misc_feature (39)..(42): n is a, c, g, or t
tcgtcggcagcgtcagatgtgtataagagacaghhhhhnnnnggagtctgccaggccctcaca

SEQ ID NO: 356 - DNA, 64 bp, Artificial Sequence
  Synthetic polynucleotide
  misc_feature (39)..(42): n is a, c, g, or t
tcgtcggcagcgtcagatgtgtataagagacaghhhhhnnnngaagtctgccagcaccaaccag

SEQ ID NO: 357 - DNA, 64 bp, Artificial Sequence
  Synthetic polynucleotide
  misc_feature (39)..(42): n is a, c, g, or t
tcgtcggcagcgtcagatgtgtataagagacaghhhhhnnnnggagtcgcccagccccaaccag

SEQ ID NO: 358 - DNA, 64 bp, Artificial Sequence
  Synthetic polynucleotide
  misc_feature (39)..(42): n is a, c, g, or t
tcgtcggcagcgtcagatgtgtataagagacaghhhhhnnnnggagtccgccagcaccaaccag

SEQ ID NO: 359 - DNA, 65 bp, Artificial Sequence
  Synthetic polynucleotide
  misc_feature (39)..(42): n is a, c, g, or t
tcgtcggcagcgtcagatgtgtataagagacaghhhhhnnnngtgagcaacatgagccctgaaga

SEQ ID NO: 360 - DNA, 65 bp, Artificial Sequence
  Synthetic polynucleotide
  misc_feature (39)..(42): n is a, c, g, or t
tcgtcggcagcgtcagatgtgtataagagacaghhhhhnnnngagttctaagaagctccttctca